European Patent Application EP 4 257 155 A2, published October 11, 2023. Title: COMPOSITIONS AND METHODS FOR TREATING WILSON'S DISEASE. Applicant: ENCODED THERAPEUTICS, INC. Application WO PCT/US2019/061808, filed November 15, 2019. The sequence listing filed with the application follows.

SEQUENCE LISTING (92 sequences)

SEQ ID NO: 1 - DNA, 4398 bp, Homo sapiens
  source 1..4398: mol_type = other DNA
atgcctgagcaggagagacagatcacagccagagaaggggccagtcggaaaatcttatctaagctttctttgcctacccgtgcctgggaaccagcaatgaagaagagttttgcttttgacaatgttggctatgaaggtggtctggatggcctgggcccttcttctcaggtggccaccagcacagtcaggatcttgggcatgacttgccagtcatgtgtgaagtccattgaggacaggatttccaatttgaaaggcatcatcagcatgaaggtttccctggaacaaggcagtgccactgtgaaatatgtgccatcggttgtgtgcctgcaacaggtttgccatcaaattggggacatgggcttcgaggccagcattgcagaaggaaaggcagcctcctggccctcaaggtccttgcctgcccaggaggctgtggtcaagctccgggtggagggcatgacctgccagtcctgtgtcagctccattgaaggcaaggtccggaaactgcaaggagtagtgagagtcaaagtctcactcagcaaccaagaggccgtcatcacttatcagccttatctcattcagcccgaagacctcagggaccatgtaaatgacatgggatttgaagctgccatcaagagcaaagtggctcccttaagcctgggaccaattgatattgagcggttacaaagcactaacccaaagagacctttatcttctgctaaccagaattttaataattctgagaccttggggcaccaaggaagccatgtggtcaccctccaactgagaatagatggaatgcattgtaagtcttgcgtcttgaatattgaagaaaatattggccagctcctaggggttcaaagtattcaagtgtccttggagaacaaaactgcccaagtaaagtatgacccttcttgtaccagcccagtggctctgcagagggctatcgaggcacttccacctgggaattttaaagtttctcttcctgatggagccgaagggagtgggacagatcacaggtcttccagttctcattcccctggctccccaccgagaaaccaggtccagggcacatgcagtaccactctgattgccattgccggcatgacctgtgcatcctgtgtccattccattgaaggcatgatctcccaactggaaggggtgcagcaaatatcggtgtctttggccgaagggactgcaacagttctttataatccctctgtaattagcccagaagaactcagagctgctatagaagacatgggatttgaggcttcagtcgtttctgaaagctgttctactaaccctcttggaaaccacagtgctgggaactccatggtgcaaactacagatggtacacctacatctgtgcaggaagtggctccccacactgggaggctccctgcaaaccatgccccggacatcttggcaaagtccccacaatcaaccagagcagtggcaccgcagaagtgcttcttacagatcaaaggcatgacctgtgcatcctgtgtgtctaacatagaaaggaatctgcagaaagaagctggtgttctctccgtgttggttgccttgatggcaggaaaggcagagatcaagtatgacccagaggtcatccagcccctcgagatagctcagttcatccaggacctgggttttgaggcagcagtcatggaggactacgcaggctccgatggcaacattgagctgacaatcacagggatgacctgcgcgtcctgtgtccacaacatagagtccaaactcacgaggacaaatggcatcacttatgcctccgttgcccttgccaccagcaaagcccttgttaagtttgacccggaaattatcggtccacgggatattatcaaaattattgaggaaattggctttcatgcttccctggcccagagaaaccccaacgctcatcacttggaccacaagatggaaataaagcagtggaagaagtctttcctgtgcagcctggtgtttggcatccctgtcatggccttaatgatctatatgctgatacccagcaacgagccccaccagtccatggtcctggaccacaacatcattccaggactgtccattctaaatctcatcttctttatcttgtgtacctttgtccagctcctcggtgggtggtacttctacgttcaggcctacaaatctctgagacacaggtcagccaacatggacgtgctcatcgtcctggccacaagcattgcttatgtttattctctggtcatcctggtggttgctgtggctgagaaggcggagaggagccctgtgacattcttcgacacgccccccatgctctttgtgttcattgccctgggccggtggctggaacacttggcaaagagcaaaacctcagaagccctggctaaactcatgtctctccaagccacagaagccaccgttgtgacccttggtgaggacaatttaatcatcagggaggagcaagtccccatggagctggtgcagcggggcgatatcgtcaaggtggtccctgggggaaagtttccagtggatgggaaagtcctggaaggcaataccatggctgatgagtccctcatcacaggagaagccatgccagtcactaagaaacccggaagcactgtaattgcggggtctataaatgcacatggctctgtgctcattaaagctacccacgtgggcaatgacaccactttggctcagattgtgaaactggtggaagaggctcagatgtcaaaggcacccattcagcagctggctgaccggtttagtggatattttgtcccatttatcatcatcatgtcaactttgacgttggtggtatggattgtaatcggttttatcgattttggtgttgttcagagatactttcctaaccccaacaagcacatctcccagacagaggtgatcatccggtttgctttccagacgtccatcacggtgctgtgcattgcctgcccctgctccctggggctggccacgcccacggctgtcatggtgggcaccggggtggccgcgcagaacggcatcctcatcaagggaggcaagcccctggagatggcgcacaagataaagactgtgatgtttgacaagactggcaccattacccatggcgtccccagggtcatgcgggtgctcctgctgggggatgtggccacactgcccctcaggaaggttctggctgtggtggggactgcggaggccagcagtgaacaccccttgggcgtggcagtcaccaaatactgtaaagaggaacttggaacagagaccttgggatactgcacggacttccaggcagtgccaggctgtggaattgggtgcaaagtcagcaacgtggaaggcatcctggcccacagtgagcgccctttgagtgcaccggccagtcacctgaatgaggctggcagccttcccgcagaaaaagatgcagtcccccagaccttctctgtgctgattggaaaccgtgagtggctgaggcgcaacggtttaaccatttctagcgatgtcagtgacgctatgacagaccacgagatgaaaggacagacagccatcctggtggctattgacggtgtgctctgtgggatgatcgcaatcgcagacgctgtcaagcaggaggctgccctggctgtgcacacgctgcagagcatgggtgtggacgtggttctgatcacgggggacaaccggaagacagccagagctattgccacccaggttggcatcaacaaagtctttgcagaggtgctgccttcgcacaaggtggccaaggtccaggagctccagaataaagggaagaaagtcgccatggtgggggatggggtcaatgactccccggccttggcccaggcagacatgggtgtggccattggcaccggcacggatgtggccatcgaggcagccgacgtcgtccttatcagaaatgatttgctggatgtggtggctagcattcacctttccaagaggactgtccgaaggatacgcatcaacctggtcctggcactgatttataacctggttgggatacccattgcagcaggtgtcttcatgcccatcggcattgtgctgcagccctggatgggctcagcggccatggcagcctcctctgtgtctgtggtgctctcatccctgcagctcaagtgctataagaagcctgacctggagaggtatgaggcacaggcgcatggccacatgaagcccctgacggcatcccaggtcagtgtgcacataggcatggatgacaggtggcgggactcccccagggccacaccatgggaccaggtcagctatgtcagccaggtgtcgctgtcctccctgacgtccgacaagccatctcggcacagcgctgcagcagacgatgatggggacaagtggtctctgctcctgaatggcagggatgaggagcagtacatctga

SEQ ID NO: 2 - protein, 1465 aa, Homo sapiens
MPEQERQITAREGASRKILSKLSLPTRAWEPAMKKSFAFDNVGYEGGLDGLGPSSQVATSTVRILGMTCQSCVKSIEDRISNLKGIISMKVSLEQGSATVKYVPSVVCLQQVCHQIGDMGFEASIAEGKAASWPSRSLPAQEAVVKLRVEGMTCQSCVSSIEGKVRKLQGVVRVKVSLSNQEAVITYQPYLIQPEDLRDHVNDMGFEAAIKSKVAPLSLGPIDIERLQSTNPKRPLSSANQNFNNSETLGHQGSHVVTLQLRIDGMHCKSCVLNIEENIGQLLGVQSIQVSLENKTAQVKYDPSCTSPVALQRAIEALPPGNFKVSLPDGAEGSGTDHRSSSSHSPGSPPRNQVQGTCSTTLIAIAGMTCASCVHSIEGMISQLEGVQQISVSLAEGTATVLYNPSVISPEELRAAIEDMGFEASVVSESCSTNPLGNHSAGNSMVQTTDGTPTSVQEVAPHTGRLPANHAPDILAKSPQSTRAVAPQKCFLQIKGMTCASCVSNIERNLQKEAGVLSVLVALMAGKAEIKYDPEVIQPLEIAQFIQDLGFEAAVMEDYAGSDGNIELTITGMTCASCVHNIESKLTRTNGITYASVALATSKALVKFDPEIIGPRDIIKIIEEIGFHASLAQRNPNAHHLDHKMEIKQWKKSFLCSLVFGIPVMALMIYMLIPSNEPHQSMVLDHNIIPGLSILNLIFFILCTFVQLLGGWYFYVQAYKSLRHRSANMDVLIVLATSIAYVYSLVILVVAVAEKAERSPVTFFDTPPMLFVFIALGRWLEHLAKSKTSEALAKLMSLQATEATVVTLGEDNLIIREEQVPMELVQRGDIVKVVPGGKFPVDGKVLEGNTMADESLITGEAMPVTKKPGSTVIAGSINAHGSVLIKATHVGNDTTLAQIVKLVEEAQMSKAPIQQLADRFSGYFVPFIIIMSTLTLVVWIVIGFIDFGVVQRYFPNPNKHISQTEVIIRFAFQTSITVLCIACPCSLGLATPTAVMVGTGVAAQNGILIKGGKPLEMAHKIKTVMFDKTGTITHGVPRVMRVLLLGDVATLPLRKVLAVVGTAEASSEHPLGVAVTKYCKEELGTETLGYCTDFQAVPGCGIGCKVSNVEGILAHSERPLSAPASHLNEAGSLPAEKDAVPQTFSVLIGNREWLRRNGLTISSDVSDAMTDHEMKGQTAILVAIDGVLCGMIAIADAVKQEAALAVHTLQSMGVDVVLITGDNRKTARAIATQVGINKVFAEVLPSHKVAKVQELQNKGKKVAMVGDGVNDSPALAQADMGVAIGTGTDVAIEAADVVLIRNDLLDVVASIHLSKRTVRRIRINLVLALIYNLVGIPIAAGVFMPIGIVLQPWMGSAAMAASSVSVVLSSLQLKCYKKPDLERYEAQAHGHMKPLTASQVSVHIGMDDRWRDSPRATPWDQVSYVSQVSLSSLTSDKPSRHSAAADDDGDKWSLLLNGRDEEQYI

SEQ ID NO: 3 - DNA, 4398 bp, synthetic construct
  source 1..4398: mol_type = other DNA; note = Description of Artificial Sequence: Syntheticpolynucleotide
atgcctgagcaggaaaggcaaatcacggcccgcgaaggggcttctcgcaagatacttagcaagctttcacttcctacgcgagcctgggaacctgccatgaagaaaagctttgcctttgataatgttggctacgagggagggcttgatggtttgggcccatccagccaggtagcaacgtcaactgttaggatcttggggatgacatgccaaagctgcgtgaagtccattgaagaccggatatccaatctcaaaggtatcattagtatgaaagtgtccctggagcagggatctgcgacagttaagtacgttccttcagtcgtgtgcctgcaacaagtctgccatcagataggcgacatggggttcgaggcctcaattgcggagggtaaggcggccagctggccatctagaagcctgcccgcacaagaggcggttgtgaaactgagggttgagggcatgacttgtcaatcttgcgtaagtagtatcgagggaaaggttcggaagctccagggagttgtgagagttaaagtgagcctctcaaatcaagaagccgttataacgtaccagccctacttgattcagcctgaggatttgcgcgaccatgtcaatgatatgggttttgaagcggctattaagagtaaggtggcccctctgagtctcgggccgattgacatcgaaaggcttcaatccacgaaccctaagagacctcttagtagtgcgaatcagaattttaacaatagtgagacgctgggtcatcaaggatctcatgtagttactttgcaactgagaattgacggcatgcattgtaaatcctgtgtgctgaacattgaggaaaatattgggcaactgcttggagtgcaaagcatacaagtctccctcgagaacaaaacggcccaggtgaagtacgacccgtcatgcacttcaccggtggccctccaaagagcgattgaggctctgcccccaggtaatttcaaagtaagcctgccggatggggctgaggggtctggaactgaccacagatcaagtagctcacacagcccaggaagcccaccgcggaaccaggttcaggggacgtgctcaacaactcttatcgctatagcgggtatgacttgtgcgtcctgtgttcattcaatcgagggaatgataagtcagcttgagggagtccagcagataagtgtttcccttgccgaggggacagctaccgtactttacaatccgagcgtgattagtcctgaagaacttcgggcagcaattgaggacatggggtttgaggcgagcgtcgtgagcgagtcatgctcaactaaccctcttggaaatcacagtgccgggaactcaatggtgcaaacgacagatgggaccccgacttctgtacaggaagtcgctccccacaccggacggcttcccgcaaaccatgccccagacattctcgcgaaatcaccgcagtcaacacgcgcggtggcgccgcagaaatgttttcttcagattaaaggcatgacgtgcgccagttgtgtatctaacatcgaacggaacttgcagaaagaagctggtgtactgagcgtgttggtagcgcttatggccggaaaggcggaaatcaagtatgatccagaggttattcagccacttgagattgcgcagttcatccaggacttgggctttgaggcagcagtgatggaagactacgccggtagtgatggtaacattgagcttaccatcacaggcatgacctgtgcaagctgtgtccacaatatcgagtctaagcttacccgaacaaacgggatcacgtatgccagcgtcgcgcttgcaacgtccaaagcattggtaaaattcgacccagaaatcataggaccccgcgatattattaagattatcgaggaaattggcttccacgcctctctggcccagcgcaacccaaacgctcatcatcttgatcataaaatggaaatcaaacagtggaagaagtctttcctttgtagtctggtcttcgggatacctgttatggcacttatgatctacatgctcattccgtctaacgagccacaccaaagtatggttttggaccataatataatacctgggctgagcattcttaacctgatcttctttatactgtgcacgtttgtacaattgcttggtggatggtatttttatgtacaggcgtataaaagcctgcggcatcgatctgccaatatggacgtactcattgtactggcgacatcaattgcctacgtgtacagtcttgtcattttggtagtagcggtcgctgaaaaagcagaacggagccctgttactttcttcgataccccgccgatgctttttgttttcattgctcttggccggtggttggagcatctggctaaatcaaaaacgagcgaggcccttgcaaagctcatgtcattgcaagcgactgaagccacggtggtcaccctgggcgaagataacttgattatcagagaagagcaagtgcccatggaactggttcaaagaggtgatatagtgaaggttgtgccgggggggaagttccccgttgatgggaaggtacttgagggtaatacaatggcagatgaatcattgataacgggagaggctatgcccgtcactaagaaacctgggtcaactgtcatcgcagggtctatcaacgcccatgggagcgtattgataaaagctacgcatgtcgggaatgatactacgttggctcagatagttaagcttgtcgaggaagctcaaatgagcaaggctcctatacagcaactggccgataggttcagtgggtatttcgtgccgttcattataataatgagtactttgacattggtagtatggattgtaatcgggttcatagactttggagtagtacagcgatactttccaaatcccaacaagcatatctcccaaaccgaggttataatcagattcgctttccaaacgtccataacggtcctctgtatagcctgtccgtgtagcttgggtcttgcaactccaacggcggtcatggttggaaccggagttgcggcccaaaacggcatactcattaagggtgggaaacctctggaaatggcacataagataaaaacagttatgtttgataagacagggaccattacccatggcgtgccgagagttatgagggtcctccttttgggtgatgttgcgactctgccccttagaaaggtattggcagtggttgggacggcggaagcgtcctcagaacacccgctgggggtagccgtaactaagtactgtaaagaagagctcggtacagagactcttgggtactgtacagatttccaagctgtcccaggttgcggaatcggatgtaaggtcagcaatgtcgaaggaatcttggctcattcagaaagacctttgtcagcacctgcatctcatttgaatgaggctggcagtttgccagctgaaaaagacgctgtaccccaaacttttagtgtcttgattggcaaccgagagtggctgcgccgcaatgggctcactataagctccgatgtatcagatgccatgacagaccacgaaatgaaaggtcagactgcgatactggtggcaatcgatggtgtactctgtggtatgatagccatagccgatgcagttaaacaggaagcagcacttgccgtacacactttgcaatctatgggtgtcgacgtagtcctgattaccggtgacaacagaaaaaccgcgagagctattgccacacaagttggcattaacaaagtgtttgctgaggttctgccttcccataaagtcgctaaagttcaggaactgcaaaataagggaaaaaaagtcgctatggttggcgacggcgtcaatgactcaccggcattggcgcaagcggatatgggcgtggcgatcggcactggcacagacgtcgcgatagaggccgcggacgtagttttgatcagaaatgatctccttgatgttgttgcctctatccatttgagcaaacgaactgtgcgaagaatccgaataaatcttgtcctcgcacttatttataatctggttggcattccaattgccgctggtgtcttcatgcctatcggaatcgtccttcagccatggatgggcagcgcggcgatggcagctagttcagtctctgtggtccttagttccctccagctgaaatgctataaaaaacctgatcttgagaggtatgaggcccaagcacatggccatatgaaaccacttacggcaagtcaggtgtcagttcacatcgggatggatgacaggtggagggattccccgcgcgccactccgtgggaccaggtaagctatgtatctcaggtttctctcagtagtttgaccagtgacaaaccttctcgacattctgctgccgcagatgacgatggtgataagtggtctcttcttcttaacgggagggacgaagagcaatacatttga

SEQ ID NO: 4 - DNA, 4398 bp, synthetic construct
  source 1..4398: mol_type = other DNA; note = Description of Artificial Sequence: Syntheticpolynucleotide
atgccagaacaggaacggcaaataacagctcgagaaggtgcttcacggaagatactgagtaaactttcattgccaacccgcgcctgggagcccgctatgaagaaatcctttgccttcgacaacgtgggatacgaggggggtttggacggacttggaccctcctctcaagtagctacatctactgttcgaattttgggaatgacatgtcaaagttgtgtcaaatctatagaggatagaatcagcaacctgaagggcatcatatcaatgaaggtctctttggaacaaggatccgcaacagtaaagtacgtacccagtgtggtatgccttcaacaggtctgccaccagataggggacatgggatttgaagcatccatcgccgaggggaaagcagcttcttggcctagccgaagcttgccagcccaggaagcagtagtgaagctcagagttgagggtatgacttgccagtcttgcgtttcctctatagagggcaaagtccgcaaactgcagggggttgtgcgcgtgaaagtaagtctgagcaaccaagaggcagtaatcacatatcaaccatatctcattcagcctgaggacttgcgagaccatgttaacgatatgggatttgaggctgccattaaatccaaagtggcacccctctctcttgggccaatagacatagagaggcttcagagtactaacccaaaacggccattgtcttcagctaatcaaaacttcaacaattccgaaaccctcggtcatcagggctcacatgttgtaactctgcagttgcgcatagacggaatgcattgcaagtcctgcgttctgaacatcgaagaaaacataggtcagcttctgggggtccagtctatacaagtgagtctcgaaaacaagactgcccaagttaaatatgatccaagctgtaccagcccagttgccctgcaaagagccatagaagcactgcctcctggaaatttcaaggtttctcttccagacggagctgaaggaagcggcactgaccatcgatcctcaagtagccatagccctggatctccccccagaaatcaagtccagggtacatgcagtaccaccctcatagccatagccggcatgacctgtgcttcatgcgtacacagtattgaaggaatgatctcccagttggagggagtacagcaaatttccgtatccttggccgaaggtactgcaactgtactctacaatccatccgttataagccccgaggaacttagagccgcaattgaggacatgggattcgaggcaagtgtagtttcagaatcatgtagtactaatccacttggtaaccattcagcaggtaacagcatggtacaaaccacagacggcactccaacatccgttcaggaagtggccccccataccggccgcctccccgccaaccacgcacctgacatcctcgctaagtccccccaatcaacacgggctgtagccccacagaagtgctttctgcagataaagggcatgacttgcgcaagctgcgtttcaaacatcgagcgaaaccttcagaaagaggccggcgtgctgagtgtcttggttgctcttatggcaggtaaagctgaaatcaaatacgatcccgaagtcatacaacctcttgaaatcgcacaatttatccaagacttgggcttcgaggctgcagtcatggaagactacgctggctcagacggcaacatcgaattgacaataaccgggatgacatgtgcttcctgcgttcataatatagagtctaagctcactagaaccaatggtattacctatgcttcagtggcactcgctacctccaaagcacttgtcaaatttgacccagagatcatagggccacgggatattatcaaaattattgaggaaataggtttccatgcatcactcgctcagaggaaccccaacgcccatcatttggatcacaaaatggaaataaaacagtggaagaaaagtttcctgtgtagccttgtgttcggcatcccagtgatggcactgatgatctacatgttgatacccagcaatgaaccacaccagagcatggttcttgatcataatattatccccggactcagcattttgaatcttatattctttattctctgcacttttgtccaactcctcggaggctggtatttttacgtccaagcctacaagagcttgaggcatagatcagctaacatggatgttttgattgttttggcaacaagtatcgcctacgtctacagtctcgtgatactggtcgtggcagttgctgaaaaagcagagcgcagtccagtaacattttttgatacacccccaatgctcttcgtatttatcgccttgggacggtggcttgagcaccttgctaaatcaaagactagcgaagctcttgccaagctcatgagtctccaagcaacagaagcaactgtggtaactctgggggaagataacctcataatacgggaggaacaagtacctatggaattggtacagcgaggggatattgtaaaagttgtccccggcgggaagtttccagtggacggcaaggtactggagggcaacactatggcagatgagagtttgatcaccggcgaagcaatgcctgtgactaaaaaaccaggaagtaccgtcattgccgggagcattaatgcacatggtagtgtcctgatcaaggccacacatgtaggcaacgatactactctggcacagatcgtgaagctcgtagaagaagcacagatgtctaaggcccccattcagcaactcgcagaccgatttagtggatacttcgttccattcataatcattatgtctacattgaccctcgttgtttggatcgtaataggcttcatagattttggagtagttcagcgatacttccccaaccctaataaacatattagtcagaccgaggttataataagatttgctttccagacttcaataaccgtactctgtatagcatgtccctgctccctgggcctcgccacccctacagctgttatggttggcaccggagtagcagcccagaacggcattttgattaaaggtggcaagcctcttgaaatggctcataaaattaaaacagtaatgttcgacaaaactgggaccatcactcacggcgtgccccgcgttatgcgagttctcttgttgggcgatgttgcaaccttgcctctgagaaaagtactcgctgtagttggtacagctgaagcttcttccgagcatccacttggcgtggcagtgactaagtattgcaaggaagaactgggtaccgagacccttggctactgtaccgattttcaggccgtgcccggctgtgggataggttgtaaggtttcaaacgtggaggggattctggcacactcagaacgcccactctctgctccagctagccatctcaacgaagcagggtcacttcccgctgaaaaggacgcagttcctcaaactttcagtgtgctgatcggtaaccgcgagtggttgcggaggaatggcttgacaatcagttccgacgtcagtgatgctatgaccgatcacgaaatgaaggggcaaactgcaatattggtggctattgacggagtgctgtgtggaatgatagctatcgctgatgctgtcaaacaagaagctgcattggccgtgcacactttgcaatctatgggcgtagatgtagtcttgatcaccggggataatcgcaagaccgcccgcgctattgccacacaggtgggaatcaacaaagtcttcgcagaggttctgccaagtcataaagtcgctaaggtacaggagctccaaaataagggcaagaaggttgccatggttggtgacggcgtcaatgattctcccgccctcgctcaggctgatatgggggtcgccatcggaaccggaactgatgttgccatcgaagccgccgacgtggttctcatacggaacgacttgttggatgtcgtggcctcaatacacctctccaaacggacagtacgccggataaggattaatttggttcttgccctgatctacaatctggtaggaatccctattgctgctggtgtgtttatgccaatagggattgtcctccaaccttggatgggatccgcagctatggccgcctcctcagtgtcagtggtgttgtcatctctccaactcaagtgttataaaaaaccagatcttgagcgatatgaggcacaagctcatggccacatgaagcctctcacagcctctcaagtttcagtgcacataggtatggatgatagatggcgggacagtcccagggctacaccttgggaccaggttagctatgtgtcacaggtgtcactgtcctcccttaccagtgataagccaagtaggcattccgccgcagctgacgatgatggcgataagtggtctcttctcctcaacggacgagatgaagaacaatacatttga

SEQ ID NO: 5 - DNA, 4398 bp, synthetic construct
  source 1..4398: mol_type = other DNA; note = Description of Artificial Sequence: Syntheticpolynucleotide
atgccagaacaggaacgccagattaccgcacgagagggagccagccggaagatcctgagcaaactgagcctgcccaccagagcttgggagcccgccatgaagaagagcttcgcctttgacaacgtgggatacgagggaggcctggatggcctgggacctagctcccaggtggccaccagcaccgtgagaatcctgggcatgacatgccagagctgcgtgaagtccatcgaggacagaatctctaatctgaagggcatcatctctatgaaggtgagcctggagcagggctccgccaccgtgaagtatgtgccttctgtggtgtgcctgcagcaggtgtgccaccagatcggcgatatgggcttcgaggccagcatcgcagagggcaaggcagcctcctggccttctcggagcctgccagcacaggaggcagtggtgaagctgagagtggaaggaatgacctgtcagagctgcgtgagcagcatcgagggcaaggtgaggaagctgcagggcgtggtgcgcgtgaaggtgtccctgtctaaccaggaggccgtgatcacctaccagccctatctgatccagcctgaggacctgagggatcacgtgaatgacatgggcttcgaggccgccatcaagagcaaggtggcaccactgtccctgggaccaatcgacatcgagcggctgcagtccaccaacccaaagcggcccctgagcagcgccaaccagaacttcaacaattctgagacactgggacaccagggcagccacgtggtgaccctgcagctgaggatcgacggcatgcactgcaagagctgcgtgctgaacatcgaggagaatatcggccagctgctgggcgtgcagtccatccaggtgtctctggagaacaagacagcccaggtgaagtacgatccttcttgcaccagcccagtggccctgcagagggcaatcgaggccctgccccctggcaatttcaaggtgtccctgcctgacggagcagagggctctggcaccgatcaccggagcagcagcagccactccccaggctctccacccagaaaccaggtgcagggcacatgttctaccacactgatcgcaatcgcaggaatgacctgcgccagctgcgtgcactccatcgagggcatgatcagccagctggagggcgtgcagcagatcagcgtgtccctggccgagggcaccgcaacagtgctgtacaatcccagcgtgatctcccctgaggagctgagggcagcaatcgaggatatgggatttgaggcctccgtggtgtctgagagctgctccacaaaccccctgggcaatcactctgccggcaacagcatggtgcagaccacagacggcacccctacaagcgtgcaggaggtggcaccacacaccggccggctgccagcaaatcacgcaccagacatcctggccaagtctccccagagcacaagagccgtggcccctcagaagtgttttctgcagatcaagggcatgacctgcgcctcctgcgtgagcaacatcgagcggaatctgcagaaggaggcaggcgtgctgtccgtgctggtggccctgatggcaggcaaggccgagatcaagtacgaccctgaagtgatccagccactggagatcgcccagttcatccaggatctgggctttgaggccgccgtgatggaggactatgccggcagcgatggcaacatcgagctgaccatcacaggcatgacctgcgcctcttgcgtgcacaacatcgagagcaagctgaccagaacaaatggcatcacatacgcctctgtggccctggccaccagcaaggccctggtgaagttcgaccccgagatcatcggcccccgggacatcatcaagatcatcgaggagatcggctttcacgcctccctggcccagcgcaacccaaatgcccaccacctggaccacaagatggagatcaagcagtggaagaagtccttcctgtgctctctggtgtttggcatccccgtgatggccctgatgatctacatgctgatcccttccaacgagccacaccagtctatggtgctggatcacaacatcatccctggcctgagcatcctgaatctgatcttctttatcctgtgcacattcgtgcagctgctgggcggctggtacttttatgtgcaggcctataagtccctgcggcaccggagcgccaatatggacgtgctgatcgtgctggccaccagcatcgcctacgtgtatagcctggtcatcctggtggtggcagtggcagagaaggcagagcggtcccccgtgaccttctttgatacacctccaatgctgttcgtgtttatcgccctgggcagatggctggagcacctggccaagagcaagacctccgaggccctggccaagctgatgagcctgcaggccacagaggccaccgtggtgacactgggcgaggacaacctgatcatcagggaggagcaggtgcctatggagctggtgcagcgcggcgacatcgtgaaggtggtgccaggcggcaagttcccagtggacggcaaggtgctggagggcaatacaatggccgatgagagcctgatcaccggcgaggccatgcctgtgaccaagaagccaggctctacagtgatcgcaggcagcatcaacgcccacggctccgtgctgatcaaggccacccacgtgggcaatgacaccacactggcccagatcgtgaagctggtggaggaggcccagatgtccaaggcccctatccagcagctggccgatcggttctccggctacttcgtgcccttcatcatcatcatgtctaccctgacactggtggtgtggatcgtgatcggcttcatcgactttggcgtggtgcagaggtattttcccaaccctaataagcacatcagccagaccgaagtgatcatccgcttcgcctttcagaccagcatcacagtgctgtgcatcgcatgcccatgttccctgggcctggccaccccaacagccgtgatggtgggcacaggcgtggcagcacagaacggcatcctgatcaagggcggcaagcccctggagatggcccacaagatcaagaccgtgatgtttgacaagaccggcacaatcacccacggcgtgcccagagtgatgagagtgctgctgctgggcgatgtggccacactgcctctgagaaaggtgctggccgtggtgggcaccgccgaggcctcctctgagcacccactgggagtggccgtgacaaagtactgcaaggaggagctgggcacagagacactgggctattgtaccgacttccaggccgtgcccggatgcggaatcggctgtaaggtgagcaacgtggagggcatcctggcacactccgagcggcccctgagcgcccctgcctcccacctgaatgaggcaggctctctgcccgccgagaaggacgccgtgcctcagaccttcagcgtgctgatcggcaacagagagtggctgcggagaaatggcctgaccatcagctccgacgtgtccgatgccatgacagatcacgagatgaagggccagaccgcaatcctggtggcaatcgacggcgtgctgtgcggcatgatcgccatcgccgatgcagtgaagcaggaggccgccctggccgtgcacaccctgcagagcatgggcgtggacgtggtgctgatcaccggcgataacaggaagacagccagagccatcgccacccaagtgggcatcaataaggtgttcgccgaggtgctgccttcccacaaggtggccaaggtgcaggagctgcagaacaagggcaagaaggtggctatggtgggcgacggcgtgaatgattctccagccctggcccaggcagacatgggagtggcaatcggcacaggcaccgacgtggcaatcgaggccgccgatgtggtgctgatcaggaatgacctgctggatgtggtggcctctatccacctgagcaagcggaccgtgaggcgcatcagaatcaacctggtgctggccctgatctacaatctggtgggcatcccaatcgccgccggcgtgtttatgccaatcggcatcgtgctgcagccctggatgggcagcgccgctatggccgcctctagcgtgagcgtggtgctgtcctctctgcagctgaagtgctacaagaagcccgacctggagcggtacgaggcacaggcccacggccacatgaagccactgaccgcctctcaggtgagcgtgcacatcggcatggacgataggtggagggacagcccaagggccacaccctgggatcaggtgagctacgtgagccaggtgagcctgagcagcctgaccagcgacaagccctcccgccacagcgccgccgccgacgacgacggggacaagtggagcctgctgctgaacgggagggatgaagaacagtacatttga

SEQ ID NO: 6 - DNA, 4398 bp, synthetic construct
  source 1..4398: mol_type = other DNA; note = Description of Artificial Sequence: Syntheticpolynucleotide
atgcccgaacaggaaagacagattactgccagggaaggagcctcacggaagattctctcaaaactctcactgcctacacgagcttgggagcccgctatgaagaagtccttcgcctttgacaacgtgggatacgagggcggactggatggcctgggacctagctcccaggtggccaccagcaccgtgagaatcctgggcatgacatgccagagctgcgtgaagtccatcgaggacagaatctctaacctgaagggaatcatctctatgaaggtgagcctggagcagggctccgccaccgtgaagtacgtgccttctgtggtgtgcctgcagcaggtgtgccaccagatcggagatatgggcttcgaggccagcatcgctgagggaaaggccgcttcctggccttctaggagcctgccagcccaggaggctgtggtgaagctgagagtggaaggtatgacctgtcagagctgcgtgagcagcatcgagggaaaggtgcggaagctgcagggagtggtgcgcgtgaaggtgtccctgtctaaccaggaggccgtgatcacctaccagccctacctgatccagcctgaggacctgagggatcacgtgaacgacatgggattcgaggccgctatcaagagcaaggtggctccactgtccctgggaccaatcgacatcgagaggctgcagtccaccaacccaaagaggcccctgagcagcgccaaccagaactttaacaactctgagacactgggacaccagggcagccacgtggtgaccctgcagctgcggatcgacggcatgcactgcaagtcttgcgtgctgaacatcgaggagaacatcggacagctgctgggcgtgcagtccatccaggtgtctctggagaacaagacagctcaggtgaagtacgatccttcttgcaccagcccagtggccctgcagagggctatcgaggctctgccccctggaaacttcaaggtgtccctgcctgacggagctgagggctctggaaccgatcacaggagcagcagcagccactccccaggatctccacccaggaaccaggtgcagggcacatgttctaccacactgatcgctatcgctggaatgacctgcgccagctgcgtgcactccatcgagggaatgatcagccagctggagggcgtgcagcagatcagcgtgtccctggctgagggaaccgccacagtgctgtacaaccccagcgtgatctcccctgaggagctgagagccgctatcgaggacatgggttttgaggccagcgtggtgtctgagagctgctccacaaacccactgggaaaccactctgccggcaacagcatggtgcagaccacagacggaacccctacatccgtgcaggaggtggctccacacaccggcaggctgccagctaaccacgctccagacatcctggccaagtctccccagagcacaagagctgtggcccctcagaagtgttttctgcagatcaagggcatgacctgcgcttcctgcgtgagcaacatcgagaggaacctgcagaaggaggctggagtgctgtccgtgctggtggccctgatggctggcaaggccgagatcaagtacgaccctgaagtgatccagccactggagatcgcccagttcatccaggatctgggctttgaggccgctgtgatggaggactacgctggaagcgatggcaacatcgagctgaccatcacaggaatgacctgcgcctcttgcgtgcacaacatcgagagcaagctgaccagaacaaacggcatcacatacgcttctgtggctctggccaccagcaaggccctggtgaagttcgaccccgagatcatcggacccagggacatcatcaagatcatcgaggagatcggctttcacgcttccctggcccagaggaacccaaacgctcaccacctggaccacaagatggagatcaagcagtggaagaagtccttcctgtgctctctggtgtttggaatccccgtgatggccctgatgatctacatgctgatcccttccaacgagccacaccagtctatggtgctggatcacaacatcatccctggcctgagcatcctgaacctgatcttctttatcctgtgcacattcgtgcagctgctgggcggatggtacttttacgtgcaggcttacaagtccctgaggcacaggagcgccaacatggacgtgctgatcgtgctggctaccagcatcgcctacgtgtacagcctggtcatcctggtggtggctgtggctgagaaggctgagaggagccccgtgaccttcttcgatacacctccaatgctgttcgtgtttatcgctctgggcagatggctggagcacctggccaagagcaagacctccgaggctctggccaagctgatgagcctgcaggctacagaggccaccgtggtgacactgggagaggacaacctgatcatccgggaggagcaggtgcctatggagctggtgcagcgcggcgacatcgtgaaggtggtgccaggcggaaagttccccgtggacggaaaggtgctggagggcaacacaatggctgatgagagcctgatcaccggcgaggccatgcctgtgaccaagaagccaggatctacagtgatcgctggcagcatcaacgcccacggcagcgtgctgatcaaggctacacacgtgggcaacgacaccacactggcccagatcgtgaagctggtggaggaggctcagatgtccaaggcccctatccagcagctggccgatcggttctccggctacttcgtgcccttcatcatcatcatgtctaccctgacactggtggtgtggatcgtgatcggattcatcgactttggcgtggtgcagcggtactttcccaaccctaacaagcacatcagccagaccgaagtgatcatccgcttcgcttttcagaccagcatcacagtgctgtgcatcgcctgcccatgttccctgggactggctacccccacagccgtgatggtgggcacaggagtggccgctcagaacggcatcctgatcaagggcggaaagcctctggagatggcccacaagatcaagaccgtgatgttcgacaagaccggaacaatcacccacggcgtgcccagagtgatgagagtgctgctgctgggcgatgtggctacactgcctctgagaaaggtgctggccgtggtgggaaccgctgaggcctcctctgagcacccactgggagtggctgtgacaaagtactgcaaggaggagctgggaacagagacactgggctactgtaccgacttccaggccgtgcccggatgcggaatcggctgtaaggtgagcaacgtggagggaatcctggctcactccgagaggcccctgagcgcccctgcctcccacctgaacgaggctggctctctgcccgctgagaaggacgccgtgcctcagaccttcagcgtgctgatcggaaacagagagtggctgaggagaaacggcctgaccatcagctccgacgtgtccgatgccatgacagatcacgagatgaagggccagaccgctatcctggtggccatcgacggagtgctgtgcggcatgatcgctatcgccgatgctgtgaagcaggaggccgctctggccgtgcacaccctgcagagcatgggagtggacgtggtgctgatcaccggcgataaccggaagacagcccgcgctatcgctacccaagtgggcatcaacaaggtgttcgctgaggtgctgccttcccacaaggtggccaaggtgcaggagctgcagaacaagggaaagaaggtggctatggtgggagacggcgtgaacgattctccagctctggcccaggctgacatgggcgtggctatcggaacaggcaccgacgtggctatcgaggccgctgatgtggtgctgatccggaacgacctgctggatgtggtggcttctatccacctgagcaagaggacagtgcggcgcatcagaatcaacctggtgctggccctgatctacaacctggtgggcatcccaatcgccgctggagtgtttatgccaatcggcatcgtgctgcagccctggatgggctctgccgctatggccgcttctagcgtgagcgtggtgctgtcctctctgcagctgaagtgttacaagaagcccgacctggagaggtacgaggctcaggctcacggacacatgaagcccctgaccgcttctcaggtgagcgtgcacatcggaatggacgatcggtggagggacagcccacgggccacaccctgggatcaggtgtcctacgtgtctcaggtgagcctgagcagcctgaccagcgacaagccctcccgccactctgccgctgccgatgacgatggtgacaagtggagtctgctgctgaacgggcgagatgaggaacagtacatttga

SEQ ID NO: 7 - DNA, 4398 bp, synthetic construct
  source 1..4398: mol_type = other DNA; note = Description of Artificial Sequence: Syntheticpolynucleotide
atgcccgaacaggagcgccagattactgccagagagggagcatccagaaaaatcctgagcaaactgtcactgcccacacgagcttgggaacccgcaatgaagaaaagcttcgcctttgacaacgtgggatacgagggaggactggatggactgggacctagctcccaggtggccacctctacagtccgaatcctgggcatgacttgccagagttgcgtgaaatcaattgaagaccggatcagtaatctgaagggaatcattagcatgaaagtgtccctggagcagggctcagccaccgtgaagtatgtccctagcgtggtctgcctgcagcaggtgtgccaccagatcggcgatatggggttcgaggcctccattgctgaagggaaagccgcttcttggcctagccggtccctgccagcacaggaagcagtggtcaagctgagagtggagggaatgacatgccagagctgcgtgagcagtatcgaaggaaaggtccgaaaactgcagggcgtggtccgggtgaaggtctctctgagtaaccaggaggccgtgattacctaccagccctatctgatccagcctgaagacctgagggatcacgtgaatgacatgggcttcgaggcagccatcaagtccaaagtggccccactgtctctggggcccattgacatcgaaagactgcagtccaccaacccaaagaggcccctgtcaagcgccaaccagaacttcaacaatagtgagaccctgggacaccagggctcacatgtggtcacactgcagctgaggattgacggcatgcactgcaagtcttgcgtgctgaacattgaggaaaatatcggccagctgctgggggtgcagtctatccaggtcagtctggagaacaagactgctcaggtgaaatacgatccttcatgcaccagcccagtggcactgcagcgcgctatcgaagcactgccccctggaaatttcaaggtgagcctgcctgacggagcagagggatccggaaccgatcacaggtcctctagttcacattccccaggatctccaccacgaaaccaggtgcagggaacatgttccaccacactgattgcaatcgccggcatgacttgcgcctcatgcgtgcacagcattgaagggatgatctctcagctggagggagtgcagcagatctcagtcagcctggccgagggcactgctaccgtgctgtacaatcccagtgtcatctcacctgaggaactgcgggctgcaattgaggacatggggttcgaagcttccgtggtctccgaatcttgcagtaccaaccccctggggaatcattccgccggaaactctatggtgcagactaccgacgggacacctacttctgtgcaggaggtcgcaccacacacaggacgcctgccagccaatcatgctcccgacatcctggccaaaagcccccagtccacccgggctgtggcacctcagaagtgttttctgcagatcaaaggcatgacctgcgcctcttgcgtgagcaacattgagcggaatctgcagaaggaagctggggtgctgagcgtgctggtcgcactgatggccggaaaggctgagatcaagtacgaccctgaagtgatccagccactggagattgcccagttcatccaggatctgggctttgaggccgctgtgatggaagactatgctgggagcgatggaaacattgaactgaccatcacaggcatgacttgtgcctcttgcgtgcacaacatcgagagtaaactgactagaaccaatgggattacctacgccagtgtggccctggctacatcaaaggctctggtgaaattcgaccccgagatcattggacctagggacatcatcaagatcattgaggaaatcggctttcacgcaagcctggcccagcgcaacccaaatgcccaccatctggaccataagatggagatcaagcagtggaagaaaagtttcctgtgctcactggtgtttggaatccccgtcatggccctgatgatctacatgctgatccctagcaacgagccacaccagtccatggtgctggatcataacatcattcctggcctgtccatcctgaatctgattttctttatcctgtgcacattcgtgcagctgctgggaggctggtacttttatgtgcaggcatataaatcactgcgacaccggagcgccaatatggacgtgctgattgtcctggcaacctctatcgcctacgtgtatagtctggtcatcctggtggtcgcagtggcagagaaggcagaacggagccccgtgactttctttgatacccctccaatgctgttcgtgtttatcgctctgggcagatggctggaacatctggcaaagtcaaaaaccagcgaggctctggcaaagctgatgagcctgcaggctaccgaagcaacagtggtcactctgggagaggacaacctgatcattcgcgaggaacaggtgcctatggaactggtccagcgaggcgacatcgtgaaggtggtcccagggggaaaattccccgtggacggcaaggtcctggaggggaatactatggccgatgaatccctgatcaccggcgaggctatgcctgtgacaaagaaaccaggatcaactgtcattgctggcagcatcaacgcacacgggtccgtgctgatcaaggccacacatgtcgggaatgacacaactctggctcagattgtgaaactggtcgaggaagcccagatgtccaaggctcctatccagcagctggccgatcggttctccggctacttcgtgcccttcatcattatcatgtctacactgactctggtggtctggattgtgatcggattcattgactttggcgtggtccagagatattttcccaaccctaataagcacatcagccagaccgaagtgatcatcaggttcgcatttcagaccagtattacagtgctgtgcatcgcctgcccatgttcactggggctggctacccccacagcagtgatggtcggaacaggggtggcagcacagaacggcatcctgatcaagggcgggaaacccctggagatggcccacaagatcaaaactgtgatgtttgacaaaactgggaccattacacatggagtgccacgcgtcatgcgagtgctgctgctgggcgatgtggcaaccctgcctctgagaaaggtcctggcagtggtcggaacagcagaggctagctccgaacacccactgggggtggccgtcacaaagtactgcaaagaggaactgggcactgagaccctggggtattgtactgacttccaggcagtgccaggatgcggaatcggatgtaaagtctctaacgtggaagggattctggctcacagtgagcggcccctgagcgcacctgcatcccatctgaatgaagcaggaagcctgccagcagagaaggacgctgtgcctcagaccttttccgtcctgatcggcaacagagaatggctgcggagaaatgggctgacaatttctagtgacgtgtccgatgccatgacagatcacgagatgaaaggccagactgcaattctggtggccatcgacggagtcctgtgcggcatgattgctatcgcagatgccgtgaagcaggaggctgcactggccgtccataccctgcagtctatgggcgtggacgtggtcctgatcaccggggataaccggaaaacagctagagcaattgccactcaagtgggcatcaataaggtgttcgctgaagtcctgcctagccacaaggtcgcaaaagtgcaggagctgcagaacaagggcaagaaagtcgccatggtgggagacggcgtgaatgatagcccagctctggcacaggcagacatgggagtcgctattgggacaggaactgacgtggcaatcgaggccgctgatgtggtcctgattaggaatgacctgctggatgtggtcgcttctattcatctgagtaagaggacagtgaggcgcattcgcatcaacctggtgctggccctgatctacaatctggtgggcatccccatcgcagcaggcgtgtttatgccaattgggatcgtcctgcagccctggatgggctcagctgcaatggccgcttcaagcgtgagcgtggtcctgtcctctctgcagctgaaatgctacaagaaaccagatctggagcggtacgaagctcaggcacacggacatatgaagcccctgaccgcttcccaggtgtctgtccacatcggcatggacgatagatggagggacagcccaagggcaactccatgggatcaggtcagttacgtgagccaggtcagcctgagttcactgaccagcgacaagccctcccgccattctgcagccgctgatgacgacggggacaagtggagcctgctgctgaacgggagggacgaagaacagtacatttga

SEQ ID NO: 8 - DNA, 4395 bp, synthetic construct
  source 1..4395: mol_type = other DNA; note = Description of Artificial Sequence: Syntheticpolynucleotide
atgcccgagcaggaaagacagatcaccgccagagagggcgccagccggaagatcctgagcaagctgagcctgcccaccagagcctgggagcccgccatgaagaagtccttcgccttcgacaacgtgggctacgagggcggcctggacggactgggaccatcttctcaggtggccacaagcaccgtgcgcatcctgggcatgacctgccagagctgcgtgaagtccatcgaggaccggatcagcaacctgaagggcatcatcagcatgaaggtgtccctggaacagggcagcgccaccgtgaaatacgtgccctctgtcgtgtgcctgcagcaggtgtgccaccagatcggcgacatgggcttcgaggcctctatcgccgagggaaaggccgcctcttggccctctagaagcctgcctgctcaggaagccgtcgtgaagctgcgggtggaagggatgacctgtcagtcctgcgtgtccagcatcgagggcaaagtgcggaagctgcagggcgtggtgcgcgtgaaagtgtctctgagcaaccaggaagctgtgatcacctaccagccctacctgatccagcccgaggacctgagggaccacgtgaacgatatgggatttgaggccgccatcaagagcaaggtggcccctctgtctctgggccccatcgacatcgagagactgcagagcaccaaccccaagcggcctctgagcagcgccaaccagaacttcaacaacagcgagacactgggccaccagggcagccacgtcgtgacactgcagctgcggatcgacggaatgcactgcaagagctgtgtgctgaacatcgaggaaaacatcggccagctgctgggagtgcagagcatccaggtgtcactggaaaacaagaccgcccaggtgaagtacgaccccagctgcacaagccccgtggccctgcagagagccattgaagctctgccccctggcaacttcaaagtgtccctgcctgacggagccgagggctccggaacagatcacagaagcagcagcagccacagccctggcagcccccctagaaatcaggtgcagggcacctgtagcaccaccctgatcgccattgccggcatgacatgcgccagctgcgtgcactctattgagggcatgatctcccagctggaaggcgtgcagcagatcagtgtgtctctggccgagggcaccgccacagtgctgtacaaccctagcgtgatcagccccgaagaactgagagccgccattgaggacatgggattcgaagccagcgtggtgtccgagagctgctccaccaaccctctgggcaatcacagcgccggcaacagcatggtgcagaccaccgacggcacccccaccagcgtgcaggaagtggccccacatacaggcagactgcccgccaatcacgcccccgatatcctggccaagagcccccagagtacaagagccgtggccccccagaagtgcttcctgcagatcaagggcatgacttgtgcctcttgtgtgtccaatatcgagcggaacctgcagaaagaggccggcgtgctgtctgtgctggtggctctgatggccggcaaggccgagatcaaatacgaccccgaagtgattcagcccctggaaatcgcccagtttatccaggacctgggctttgaagccgccgtgatggaagattacgccggctccgacggcaacatcgagctgaccatcaccggaatgacctgcgcctcctgtgtgcacaacattgagtccaagctgacccggaccaacggcatcacctacgcctctgtggctctggccacctccaaggccctcgtgaagttcgatcccgagatcatcggccccagggacatcatcaagatcatcgaagagatcggcttccacgccagcctggcccagaggaaccctaacgcccaccacctggaccacaagatggaaatcaagcagtggaagaaaagcttcctgtgcagcctggtgttcggcatccccgtgatggccctgatgatctacatgctgatccccagcaacgagccccaccagtccatggtgctggatcacaacatcatccccggcctgtctatcctgaacctgatcttcttcatcctgtgcaccttcgtgcagctgctgggcggctggtacttctacgtgcaggcctacaagtccctgcggcacagatccgccaacatggacgtgctgatcgtgctggccacatctatcgcctacgtgtactccctcgtgatcctggtggtggccgtggccgagaaagccgagagaagccctgtgaccttcttcgacaccccccctatgctgttcgtgtttatcgccctgggccggtggctggaacacctggccaaaagcaagaccagcgaggccctggctaagctgatgagtctgcaggccaccgaggccacagtcgtgaccctgggcgaggacaacctgatcatccgcgaggaacaggtgccaatggaactggtgcagcggggcgacatcgtgaaggtggtgcctggcggcaagttccccgtggacggaaaagtgctggaagggaataccatggccgacgagagcctgatcacaggcgaggccatgcccgtgaccaagaaacctggcagcacagtgatcgccggcagcatcaatgcccacggcagcgtgctgattaaggccacacacgtgggcaacgataccaccctggctcagattgtgaagctggtggaagaggcccagatgagcaaggcccccattcagcagctggctgaccggttcagcggctacttcgtgccctttatcatcatcatgagcaccctgacactggtcgtgtggatcgtgatcggctttatcgacttcggagtggtgcagagatacttccccaaccctaacaagcacatcagccagacagaagtgatcatcagattcgcctttcagaccagcatcaccgtgctgtgtatcgcctgcccctgtagcctgggactggccacacctaccgctgtgatggtgggaacaggcgtggccgctcagaacggcatcctgatcaaggggggcaagcctctggaaatggctcacaagatcaagaccgtgatgttcgacaagaccggcaccatcacccacggcgtgcccagagtgatgagagtgctgctgctgggggatgtggccaccctgcctctgagaaaggtgctggctgtcgtgggcacagccgaggctagctctgaacacccactgggagtggccgtgacaaagtactgcaaagaggaactgggcaccgaaaccctgggctactgcaccgactttcaggccgtgcctggctgtggcatcggctgcaaggtgtccaacgtggaaggcatcctggcccacagcgagaggccactgtctgcccctgccagccacctgaacgaggccggatctctgcccgccgaaaaggacgctgtgccccagaccttctctgtgctgattggcaacagagagtggctgcggcggaacggcctgaccatctcctccgatgtgtccgacgccatgaccgaccacgagatgaagggccagaccgccattctggtggccattgacggggtgctgtgcggcatgatcgcaatcgccgatgccgtgaaacaggaagcagcactggccgtgcacaccctgcagtctatgggagtggatgtggtgctgatcaccggcgacaacagaaagaccgccagggccattgccacccaggtgggcatcaacaaggtgttcgccgaggtgctgcccagccacaaagtggccaaggtgcaggaactgcagaacaaaggcaaaaaggtggccatggtgggagatggcgtgaacgactctcctgctctggcccaggcagatatgggcgtggccatcggcacaggcaccgacgtggcaattgaggctgctgacgtggtgctgattcggaacgacctgctggacgtggtggcctccatccacctgtccaagagaaccgtgcggcggatcagaatcaacctggtgctggcactgatctataacctcgtgggcatccctatcgccgctggcgtgttcatgcctatcggaatcgtgctgcagccctggatgggctctgccgccatggctgcaagctccgtgtctgtggtgctgtccagcctgcagctgaagtgctacaagaagcccgacctggaaagatacgaggcccaggcccacggacacatgaagcctctgacagcctcccaggtgtccgtgcacatcggcatggacgacagatggcgggacagccctagagccaccccttgggatcaggtgtcatacgtgtcacaggtgtccctgagcagcctgaccagcgacaagcccagcagacatagcgccgctgccgacgacgatggggacaagtggtccctgctgctgaacggccgggatgaggaacagtacatc

SEQ ID NO: 9 - DNA, 3966 bp, synthetic construct
  source 1..3966: mol_type = other DNA; note = Description of Artificial Sequence: Syntheticpolynucleotide
atgcccgagcaggaaagacagatcaccgccagagagggcgccagccggaagatcctgagcaagctgagcctgcccaccagagcctgggagcccgccatgaagaagtccttcgccttcgacaacgtgggctacgagggcggcctggacggactgggaccatcttctcaggtggccacaagcaccgtgcgcgaggccgccatcaagagcaaggtggcccctctgtctctgggccccatcgacatcgagagactgcagagcaccaaccccaagcggcctctgagcagcgccaaccagaacttcaacaacagcgagacactgggccaccagggcagccacgtcgtgacactgcagctgcggatcgacggaatgcactgcaagagctgtgtgctgaacatcgaggaaaacatcggccagctgctgggagtgcagagcatccaggtgtcactggaaaacaagaccgcccaggtgaagtacgaccccagctgcacaagccccgtggccctgcagagagccattgaagctctgccccctggcaacttcaaagtgtccctgcctgacggagccgagggctccggaacagatcacagaagcagcagcagccacagccctggcagcccccctagaaatcaggtgcagggcacctgtagcaccaccctgatcgccattgccggcatgacatgcgccagctgcgtgcactctattgagggcatgatctcccagctggaaggcgtgcagcagatcagtgtgtctctggccgagggcaccgccacagtgctgtacaaccctagcgtgatcagccccgaagaactgagagccgccattgaggacatgggattcgaagccagcgtggtgtccgagagctgctccaccaaccctctgggcaatcacagcgccggcaacagcatggtgcagaccaccgacggcacccccaccagcgtgcaggaagtggccccacatacaggcagactgcccgccaatcacgcccccgatatcctggccaagagcccccagagtacaagagccgtggccccccagaagtgcttcctgcagatcaagggcatgacttgtgcctcttgtgtgtccaatatcgagcggaacctgcagaaagaggccggcgtgctgtctgtgctggtggctctgatggccggcaaggccgagatcaaatacgaccccgaagtgattcagcccctggaaatcgcccagtttatccaggacctgggctttgaagccgccgtgatggaagattacgccggctccgacggcaacatcgagctgaccatcaccggaatgacctgcgcctcctgtgtgcacaacattgagtccaagctgacccggaccaacggcatcacctacgcctctgtggctctggccacctccaaggccctcgtgaagttcgatcccgagatcatcggccccagggacatcatcaagatcatcgaagagatcggcttccacgccagcctggcccagaggaaccctaacgcccaccacctggaccacaagatggaaatcaagcagtggaagaaaagcttcctgtgcagcctggtgttcggcatccccgtgatggccctgatgatctacatgctgatccccagcaacgagccccaccagtccatggtgctggatcacaacatcatccccggcctgtctatcctgaacctgatcttcttcatcctgtgcaccttcgtgcagctgctgggcggctggtacttctacgtgcaggcctacaagtccctgcggcacagatccgccaacatggacgtgctgatcgtgctggccacatctatcgcctacgtgtactccctcgtgatcctggtggtggccgtggccgagaaagccgagagaagccctgtgaccttcttcgacaccccccctatgctgttcgtgtttatcgccctgggccggtggctggaacacctggccaaaagcaagaccagcgaggccctggctaagctgatgagtctgcaggccaccgaggccacagtcgtgaccctgggcgaggacaacctgatcatccgcgaggaacaggtgccaatggaactggtgcagcggggcgacatcgtgaaggtggtgcctggcggcaagttccccgtggacggaaaagtgctggaagggaataccatggccgacgagagcctgatcacaggcgaggccatgcccgtgaccaagaaacctggcagcacagtgatcgccggcagcatcaatgcccacggcagcgtgctgattaaggccacacacgtgggcaacgataccaccctggctcagattgtgaagctggtggaagaggcccagatgagcaaggcccccattcagcagctggctgaccggttcagcggctacttcgtgccctttatcatcatcatgagcaccctgacactggtcgtgtggatcgtgatcggctttatcgacttcggagtggtgcagagatacttccccaaccctaacaagcacatcagccagacagaagtgatcatcagattcgcctttcagaccagcatcaccgtgctgtgtatcgcctgcccctgtagcctgggactggccacacctaccgctgtgatggtgggaacaggcgtggccgctcagaacggcatcctgatcaaggggggcaagcctctggaaatggctcacaagatcaagaccgtgatgttcgacaagaccggcaccatcacccacggcgtgcccagagtgatgagagtgctgctgctgggggatgtggccaccctgcctctgagaaaggtgctggctgtcgtgggcacagccgaggctagctctgaacacccactgggagtggccgtgacaaagtactgcaaagaggaactgggcaccgaaaccctgggctactgcaccgactttcaggccgtgcctggctgtggcatcggctgcaaggtgtccaacgtggaaggcatcctggcccacagcgagaggccactgtctgcccctgccagccacctgaacgaggccggatctctgcccgccgaaaaggacgctgtgccccagaccttctctgtgctgattggcaacagagagtggctgcggcggaacggcctgaccatctcctccgatgtgtccgacgccatgaccgaccacgagatgaagggccagaccgccattctggtggccattgacggggtgctgtgcggcatgatcgcaatcgccgatgccgtgaaacaggaagcagcactggccgtgcacaccctgcagtctatgggagtggatgtggtgctgatcaccggcgacaacagaaagaccgccagggccattgccacccaggtgggcatcaacaaggtgttcgccgaggtgctgcccagccacaaagtggccaaggtgcaggaactgcagaacaaaggcaaaaaggtggccatggtgggagatggcgtgaacgactctcctgctctggcccaggcagatatgggcgtggccatcggcacaggcaccgacgtggcaattgaggctgctgacgtggtgctgattcggaacgacctgctggacgtggtggcctccatccacctgtccaagagaaccgtgcggcggatcagaatcaacctggtgctggcactgatctataacctcgtgggcatccctatcgccgctggcgtgttcatgcctatcggaatcgtgctgcagccctggatgggctctgccgccatggctgcaagctccgtgtctgtggtgctgtccagcctgcagctgaagtgctacaagaagcccgacctggaaagatacgaggcccaggcccacggacacatgaagcctctgacagcctcccaggtgtccgtgcacatcggcatggacgacagatggcgggacagccctagagccaccccttgggatcaggtgtcatacgtgtcacaggtgtccctgagcagcctgaccagcgacaagcccagcagacatagcgccgctgccgacgacgatggggacaagtggtccctgctgctgaacggccgggatgaggaacagtacatc

SEQ ID NO: 10 - DNA, 3360 bp, synthetic construct
  source 1..3360: mol_type = other DNA; note = Description of Artificial Sequence: Syntheticpolynucleotide
atgcccgagcaggaaagacagatcaccgccagagagggcgccagccggaagatcctgagcaagctgagcctgcccaccagagcctgggagcccgccatgaagaagtccttcgccttcgacaacgtgggctacgagggcggcctggacggactgggaccatcttctcaggtggccacaagcaccgtgcgcagccccgaagaactgagagccgccattgaggacatgggattcgaagccagcgtggtgtccgagagctgctccaccaaccctctgggcaatcacagcgccggcaacagcatggtgcagaccaccgacggcacccccaccagcgtgcaggaagtggccccacatacaggcagactgcccgccaatcacgcccccgatatcctggccaagagcccccagagtacaagagccgtggccccccagaagtgcttcctgcagatcaagggcatgacttgtgcctcttgtgtgtccaatatcgagcggaacctgcagaaagaggccggcgtgctgtctgtgctggtggctctgatggccggcaaggccgagatcaaatacgaccccgaagtgattcagcccctggaaatcgcccagtttatccaggacctgggctttgaagccgccgtgatggaagattacgccggctccgacggcaacatcgagctgaccatcaccggaatgacctgcgcctcctgtgtgcacaacattgagtccaagctgacccggaccaacggcatcacctacgcctctgtggctctggccacctccaaggccctcgtgaagttcgatcccgagatcatcggccccagggacatcatcaagatcatcgaagagatcggcttccacgccagcctggcccagaggaaccctaacgcccaccacctggaccacaagatggaaatcaagcagtggaagaaaagcttcctgtgcagcctggtgttcggcatccccgtgatggccctgatgatctacatgctgatccccagcaacgagccccaccagtccatggtgctggatcacaacatcatccccggcctgtctatcctgaacctgatcttcttcatcctgtgcaccttcgtgcagctgctgggcggctggtacttctacgtgcaggcctacaagtccctgcggcacagatccgccaacatggacgtgctgatcgtgctggccacatctatcgcctacgtgtactccctcgtgatcctggtggtggccgtggccgagaaagccgagagaagccctgtgaccttcttcgacaccccccctatgctgttcgtgtttatcgccctgggccggtggctggaacacctggccaaaagcaagaccagcgaggccctggctaagctgatgagtctgcaggccaccgaggccacagtcgtgaccctgggcgaggacaacctgatcatccgcgaggaacaggtgccaatggaactggtgcagcggggcgacatcgtgaaggtggtgcctggcggcaagttccccgtggacggaaaagtgctggaagggaataccatggccgacgagagcctgatcacaggcgaggccatgcccgtgaccaagaaacctggcagcacagtgatcgccggcagcatcaatgcccacggcagcgtgctgattaaggccacacacgtgggcaacgataccaccctggctcagattgtgaagctggtggaagaggcccagatgagcaaggcccccattcagcagctggctgaccggttcagcggctacttcgtgccctttatcatcatcatgagcaccctgacactggtcgtgtggatcgtgatcggctttatcgacttcggagtggtgcagagatacttccccaaccctaacaagcacatcagccagacagaagtgatcatcagattcgcctttcagaccagcatcaccgtgctgtgtatcgcctgcccctgtagcctgggactggccacacctaccgctgtgatggtgggaacaggcgtggccgctcagaacggcatcctgatcaaggggggcaagcctctggaaatggctcacaagatcaagaccgtgatgttcgacaagaccggcaccatcacccacggcgtgcccagagtgatgagagtgctgctgctgggggatgtggccaccctgcctctgagaaaggtgctggctgtcgtgggcacagccgaggctagctctgaacacccactgggagtggccgtgacaaagtactgcaaagaggaactgggcaccgaaaccctgggctactgcaccgactttcaggccgtgcctggctgtggcatcggctgcaaggtgtccaacgtggaaggcatcctggcccacagcgagaggccactgtctgcccctgccagccacctgaacgaggccggatctctgcccgccgaaaaggacgctgtgccccagaccttctctgtgctgattggcaacagagagtggctgcggcggaacggcctgaccatctcctccgatgtgtccgacgccatgaccgaccacgagatgaagggccagaccgccattctggtggccattgacggggtgctgtgcggcatgatcgcaatcgccgatgccgtgaaacaggaagcagcactggccgtgcacaccctgcagtctatgggagtggatgtggtgctgatcaccggcgacaacagaaagaccgccagggccattgccacccaggtgggcatcaacaaggtgttcgccgaggtgctgcccagccacaaagtggccaaggtgcaggaactgcagaacaaaggcaaaaaggtggccatggtgggagatggcgtgaacgactctcctgctctggcccaggcagatatgggcgtggccatcggcacaggcaccgacgtggcaattgaggctgctgacgtggtgctgattcggaacgacctgctggacgtggtggcctccatccacctgtccaagagaaccgtgcggcggatcagaatcaacctggtgctggcactgatctataacctcgtgggcatccctatcgccgctggcgtgttcatgcctatcggaatcgtgctgcagccctggatgggctctgccgccatggctgcaagctccgtgtctgtggtgctgtccagcctgcagctgaagtgctacaagaagcccgacctggaaagatacgaggcccaggcccacggacacatgaagcctctgacagcctcccaggtgtccgtgcacatcggcatggacgacagatggcgggacagccctagagccaccccttgggatcaggtgtcatacgtgtcacaggtgtccctgagcagcctgaccagcgacaagcccagcagacatagcgccgctgccgacgacgatggggacaagtggtccctgctgctgaacggccgggatgaggaacagtacatc

SEQ ID NO: 11 - DNA, 2967 bp, synthetic construct
  source 1..2967: mol_type = other DNA; note = Description of Artificial Sequence: Syntheticpolynucleotide
atgcccgagcaggaaagacagatcaccgccagagagggcgccagccggaagatcctgagcaagctgagcctgcccaccagagcctgggagcccgccatgaagaagtccttcgccttcgacaacgtgggctacgagggcggcctggacggactgggaccatcttctcaggtggccacaagcaccgtgcgcctggaaatcgcccagtttatccaggacctgggctttgaagccgccgtgatggaagattacgccggctccgacggcaacatcgagctgaccatcaccggaatgacctgcgcctcctgtgtgcacaacattgagtccaagctgacccggaccaacggcatcacctacgcctctgtggctctggccacctccaaggccctcgtgaagttcgatcccgagatcatcggccccagggacatcatcaagatcatcgaagagatcggcttccacgccagcctggcccagaggaaccctaacgcccaccacctggaccacaagatggaaatcaagcagtggaagaaaagcttcctgtgcagcctggtgttcggcatccccgtgatggccctgatgatctacatgctgatccccagcaacgagccccaccagtccatggtgctggatcacaacatcatccccggcctgtctatcctgaacctgatcttcttcatcctgtgcaccttcgtgcagctgctgggcggctggtacttctacgtgcaggcctacaagtccctgcggcacagatccgccaacatggacgtgctgatcgtgctggccacatctatcgcctacgtgtactccctcgtgatcctggtggtggccgtggccgagaaagccgagagaagccctgtgaccttcttcgacaccccccctatgctgttcgtgtttatcgccctgggccggtggctggaacacctggccaaaagcaagaccagcgaggccctggctaagctgatgagtctgcaggccaccgaggccacagtcgtgaccctgggcgaggacaacctgatcatccgcgaggaacaggtgccaatggaactggtgcagcggggcgacatcgtgaaggtggtgcctggcggcaagttccccgtggacggaaaagtgctggaagggaataccatggccgacgagagcctgatcacaggcgaggccatgcccgtgaccaagaaacctggcagcacagtgatcgccggcagcatcaatgcccacggcagcgtgctgattaaggccacacacgtgggcaacgataccaccctggctcagattgtgaagctggtggaagaggcccagatgagcaaggcccccattcagcagctggctgaccggttcagcggctacttcgtgccctttatcatcatcatgagcaccctgacactggtcgtgtggatcgtgatcggctttatcgacttcggagtggtgcagagatacttccccaaccctaacaagcacatcagccagacagaagtgatcatcagattcgcctttcagaccagcatcaccgtgctgtgtatcgcctgcccctgtagcctgggactggccacacctaccgctgtgatggtgggaacaggcgtggccgctcagaacggcatcctgatcaaggggggcaagcctctggaaatggctcacaagatcaagaccgtgatgttcgacaagaccggcaccatcacccacggcgtgcccagagtgatgagagtgctgctgctgggggatgtggccaccctgcctctgagaaaggtgctggctgtcgtgggcacagccgaggctagctctgaacacccactgggagtggccgtgacaaagtactgcaaagaggaactgggcaccgaaaccctgggctactgcaccgactttcaggccgtgcctggctgtggcatcggctgcaaggtgtccaacgtggaaggcatcctggcccacagcgagaggccactgtctgcccctgccagccacctgaacgaggccggatctctgcccgccgaaaaggacgctgtgccccagaccttctctgtgctgattggcaacagagagtggctgcggcggaacggcctgaccatctcctccgatgtgtccgacgccatgaccgaccacgagatgaagggccagaccgccattctggtggccattgacggggtgctgtgcggcatgatcgcaatcgccgatgccgtgaaacaggaagcagcactggccgtgcacaccctgcagtctatgggagtggatgtggtgctgatcaccggcgacaacagaaagaccgccagggccattgccacccaggtgggcatcaacaaggtgttcgccgaggtgctgcccagccacaaagtggccaaggtgcaggaactgcagaacaaaggcaaaaaggtggccatggtgggagatggcgtgaacgactctcctgctctggcccaggcagatatgggcgtggccatcggcacaggcaccgacgtggcaattgaggctgctgacgtggtgctgattcggaacgacctgctggacgtggtggcctccatccacctgtccaagagaaccgtgcggcggatcagaatcaacctggtgctggcactgatctataacctcgtgggcatccctatcgccgctggcgtgttcatgcctatcggaatcgtgctgcagccctggatgggctctgccgccatggctgcaagctccgtgtctgtggtgctgtccagcctgcagctgaagtgctacaagaagcccgacctggaaagatacgaggcccaggcccacggacacatgaagcctctgacagcctcccaggtgtccgtgcacatcggcatggacgacagatggcgggacagccctagagccaccccttgggatcaggtgtcatacgtgtcacaggtgtccctgagcagcctgaccagcgacaagcccagcagacatagcgccgctgccgacgacgatggggacaagtggtccctgctgctgaacggccgggatgaggaacagtacatc

SEQ ID NO: 12 - DNA, 4284 bp, synthetic construct
  source 1..4284: mol_type = other DNA; note = Description of Artificial Sequence: Syntheticpolynucleotide
atgcccgagcaggaaagacagatcaccgccagagagggcgccagccggaagatcctgagcaagctgagcctgcccaccagagcctgggagcccgccatgaagaagtccttcgccttcgacaacgtgggctacgagggcggcctggacggactgggaccatcttctcaggtggccacaagcaccgtgcgcaaatacgtgccctctgtcgtgtgcctgcagcaggtgtgccaccagatcggcgacatgggcttcgaggcctctatcgccgagggaaaggccgcctcttggccctctagaagcctgcctgctcaggaagccgtcgtgaagctgcgggtggaagggatgacctgtcagtcctgcgtgtccagcatcgagggcaaagtgcggaagctgcagggcgtggtgcgcgtgaaagtgtctctgagcaaccaggaagctgtgatcacctaccagccctacctgatccagcccgaggacctgagggaccacgtgaacgatatgggatttgaggccgccatcaagagcaaggtggcccctctgtctctgggccccatcgacatcgagagactgcagagcaccaaccccaagcggcctctgagcagcgccaaccagaacttcaacaacagcgagacactgggccaccagggcagccacgtcgtgacactgcagctgcggatcgacggaatgcactgcaagagctgtgtgctgaacatcgaggaaaacatcggccagctgctgggagtgcagagcatccaggtgtcactggaaaacaagaccgcccaggtgaagtacgaccccagctgcacaagccccgtggccctgcagagagccattgaagctctgccccctggcaacttcaaagtgtccctgcctgacggagccgagggctccggaacagatcacagaagcagcagcagccacagccctggcagcccccctagaaatcaggtgcagggcacctgtagcaccaccctgatcgccattgccggcatgacatgcgccagctgcgtgcactctattgagggcatgatctcccagctggaaggcgtgcagcagatcagtgtgtctctggccgagggcaccgccacagtgctgtacaaccctagcgtgatcagccccgaagaactgagagccgccattgaggacatgggattcgaagccagcgtggtgtccgagagctgctccaccaaccctctgggcaatcacagcgccggcaacagcatggtgcagaccaccgacggcacccccaccagcgtgcaggaagtggccccacatacaggcagactgcccgccaatcacgcccccgatatcctggccaagagcccccagagtacaagagccgtggccccccagaagtgcttcctgcagatcaagggcatgacttgtgcctcttgtgtgtccaatatcgagcggaacctgcagaaagaggccggcgtgctgtctgtgctggtggctctgatggccggcaaggccgagatcaaatacgaccccgaagtgattcagcccctggaaatcgcccagtttatccaggacctgggctttgaagccgccgtgatggaagattacgccggctccgacggcaacatcgagctgaccatcaccggaatgacctgcgcctcctgtgtgcacaacattgagtccaagctgacccggaccaacggcatcacctacgcctctgtggctctggccacctccaaggccctcgtgaagttcgatcccgagatcatcggccccagggacatcatcaagatcatcgaagagatcggcttccacgccagcctggcccagaggaaccctaacgcccaccacctggaccacaagatggaaatcaagcagtggaagaaaagcttcctgtgcagcctggtgttcggcatccccgtgatggccctgatgatctacatgctgatccccagcaacgagccccaccagtccatggtgctggatcacaacatcatccccggcctgtctatcctgaacctgatcttcttcatcctgtgcaccttcgtgcagctgctgggcggctggtacttctacgtgcaggcctacaagtccctgcggcacagatccgccaacatggacgtgctgatcgtgctggccacatctatcgcctacgtgtactccctcgtgatcctggtggtggccgtggccgagaaagccgagagaagccctgtgaccttcttcgacaccccccctatgctgttcgtgtttatcgccctgggccggtggctggaacacctggccaaaagcaagaccagcgaggccctggctaagctgatgagtctgcaggccaccgaggccacagtcgtgaccctgggcgaggacaacctgatcatccgcgaggaacaggtgccaatggaactggtgcagcggggcgacatcgtgaaggtggtgcctggcggcaagttccccgtggacggaaaagtgctggaagggaataccatggccgacgagagcctgatcacaggcgaggccatgcccgtgaccaagaaacctggcagcacagtgatcgccggcagcatcaatgcccacggcagcgtgctgattaaggccacacacgtgggcaacgataccaccctggctcagattgtgaagctggtggaagaggcccagatgagcaaggcccccattcagcagctggctgaccggttcagcggctacttcgtgccctttatcatcatcatgagcaccctgacactggtcgtgtggatcgtgatcggctttatcgacttcggagtggtgcagagatacttccccaaccctaacaagcacatcagccagacagaagtgatcatcagattcgcctttcagaccagcatcaccgtgctgtgtatcgcctgcccctgtagcctgggactggccacacctaccgctgtgatggtgggaacaggcgtggccgctcagaacggcatcctgatcaaggggggcaagcctctggaaatggctcacaagatcaagaccgtgatgttcgacaagaccggcaccatcacccacggcgtgcccagagtgatgagagtgctgctgctgggggatgtggccaccctgcctctgagaaaggtgctggctgtcgtgggcacagccgaggctagctctgaacacccactgggagtggccgtgacaaagtactgcaaagaggaactgggcaccgaaaccctgggctactgcaccgactttcaggccgtgcctggctgtggcatcggctgcaaggtgtccaacgtggaaggcatcctggcccacagcgagaggccactgtctgcccctgccagccacctgaacgaggccggatctctgcccgccgaaaaggacgctgtgccccagaccttctctgtgctgattggcaacagagagtggctgcggcggaacggcctgaccatctcctccgatgtgtccgacgccatgaccgaccacgagatgaagggccagaccgccattctggtggccattgacggggtgctgtgcggcatgatcgcaatcgccgatgccgtgaaacaggaagcagcactggccgtgcacaccctgcagtctatgggagtggatgtggtgctgatcaccggcgacaacagaaagaccgccagggccattgccacccaggtgggcatcaacaaggtgttcgccgaggtgctgcccagccacaaagtggccaaggtgcaggaactgcagaacaaaggcaaaaaggtggccatggtgggagatggcgtgaacgactctcctgctctggcccaggcagatatgggcgtggccatcggcacaggcaccgacgtggcaattgaggctgctgacgtggtgctgattcggaacgacctgctggacgtggtggcctccatccacctgtccaagagaaccgtgcggcggatcagaatcaacctggtgctggcactgatctataacctcgtgggcatccctatcgccgctggcgtgttcatgcctatcggaatcgtgctgcagccctggatgggctctgccgccatggctgcaagctccgtgtctgtggtgctgtccagcctgcagctgaagtgctacaagaagcccgacctggaaagatacgaggcccaggcccacggacacatgaagcctctgacagcctcccaggtgtccgtgcacatcggcatggacgacagatggcgggacagccctagagccaccccttgggatcaggtgtcatacgtgtcacaggtgtccctgagcagcctgaccagcgacaagcccagcagacatagcgccgctgccgacgacgatggggacaagtggtccctgctgctgaacggccgggatgaggaacagtacatc

SEQ ID NO: 13 - DNA, 4215 bp, synthetic construct
  source 1..4215: mol_type = other DNA; note = Description of Artificial Sequence: Syntheticpolynucleotide
atgcccgagcaggaaagacagatcaccgccagagagggcgccagccggaagatcctgagcaagctgagcctgcccaccagagcctgggagcccgccatgaagaagtccttcgccttcgacaacgtgggctacgagggcggcctggacggactgggaccatcttctcaggtggccacaagcaccgtgcgcatcctgggcatgacctgccagagctgcgtgaagtccatcgaggaccggatcagcaacctgaagggcatcatcagcatgaaggtgtccctggaacagggcagcgccaccgtgaaatacgtgccctctgtcgtgtgcctgcagcaggtgtgccaccagatcggcgacatgggcttcgaggcctctatcgccgagggaaaggccgcctcttggccctctagaagcctgcctgctcaggaagccgtcgtgaaggaggccgccatcaagagcaaggtggcccctctgtctctgggccccatcgacatcgagagactgcagagcaccaaccccaagcggcctctgagcagcgccaaccagaacttcaacaacagcgagacactgggccaccagggcagccacgtcgtgacactgcagctgcggatcgacggaatgcactgcaagagctgtgtgctgaacatcgaggaaaacatcggccagctgctgggagtgcagagcatccaggtgtcactggaaaacaagaccgcccaggtgaagtacgaccccagctgcacaagccccgtggccctgcagagagccattgaagctctgccccctggcaacttcaaagtgtccctgcctgacggagccgagggctccggaacagatcacagaagcagcagcagccacagccctggcagcccccctagaaatcaggtgcagggcacctgtagcaccaccctgatcgccattgccggcatgacatgcgccagctgcgtgcactctattgagggcatgatctcccagctggaaggcgtgcagcagatcagtgtgtctctggccgagggcaccgccacagtgctgtacaaccctagcgtgatcagccccgaagaactgagagccgccattgaggacatgggattcgaagccagcgtggtgtccgagagctgctccaccaaccctctgggcaatcacagcgccggcaacagcatggtgcagaccaccgacggcacccccaccagcgtgcaggaagtggccccacatacaggcagactgcccgccaatcacgcccccgatatcctggccaagagcccccagagtacaagagccgtggccccccagaagtgcttcctgcagatcaagggcatgacttgtgcctcttgtgtgtccaatatcgagcggaacctgcagaaagaggccggcgtgctgtctgtgctggtggctctgatggccggcaaggccgagatcaaatacgaccccgaagtgattcagcccctggaaatcgcccagtttatccaggacctgggctttgaagccgccgtgatggaagattacgccggctccgacggcaacatcgagctgaccatcaccggaatgacctgcgcctcctgtgtgcacaacattgagtccaagctgacccggaccaacggcatcacctacgcctctgtggctctggccacctccaaggccctcgtgaagttcgatcccgagatcatcggccccagggacatcatcaagatcatcgaagagatcggcttccacgccagcctggcccagaggaaccctaacgcccaccacctggaccacaagatggaaatcaagcagtggaagaaaagcttcctgtgcagcctggtgttcggcatccccgtgatggccctgatgatctacatgctgatccccagcaacgagccccaccagtccatggtgctggatcacaacatcatccccggcctgtctatcctgaacctgatcttcttcatcctgtgcaccttcgtgcagctgctgggcggctggtacttctacgtgcaggcctacaagtccctgcggcacagatccgccaacatggacgtgctgatcgtgctggccacatctatcgcctacgtgtactccctcgtgatcctggtggtggccgtggccgagaaagccgagagaagccctgtgaccttcttcgacaccccccctatgctgttcgtgtttatcgccctgggccggtggctggaacacctggccaaaagcaagaccagcgaggccctggctaagctgatgagtctgcaggccaccgaggccacagtcgtgaccctgggcgaggacaacctgatcatccgcgaggaacaggtgccaatggaactggtgcagcggggcgacatcgtgaaggtggtgcctggcggcaagttccccgtggacggaaaagtgctggaagggaataccatggccgacgagagcctgatcacaggcgaggccatgcccgtgaccaagaaacctggcagcacagtgatcgccggcagcatcaatgcccacggcagcgtgctgattaaggccacacacgtgggcaacgataccaccctggctcagattgtgaagctggtggaagaggcccagatgagcaaggcccccattcagcagctggctgaccggttcagcggctacttcgtgccctttatcatcatcatgagcaccctgacactggtcgtgtggatcgtgatcggctttatcgacttcggagtggtgcagagatacttccccaaccctaacaagcacatcagccagacagaagtgatcatcagattcgcctttcagaccagcatcaccgtgctgtgtatcgcctgcccctgtagcctgggactggccacacctaccgctgtgatggtgggaacaggcgtggccgctcagaacggcatcctgatcaaggggggcaagcctctggaaatggctcacaagatcaagaccgtgatgttcgacaagaccggcaccatcacccacggcgtgcccagagtgatgagagtgctgctgctgggggatgtggccaccctgcctctgagaaaggtgctggctgtcgtgggcacagccgaggctagctctgaacacccactgggagtggccgtgacaaagtactgcaaagaggaactgggcaccgaaaccctgggctactgcaccgactttcaggccgtgcctggctgtggcatcggctgcaaggtgtccaacgtggaaggcatcctggcccacagcgagaggccactgtctgcccctgccagccacctgaacgaggccggatctctgcccgccgaaaaggacgctgtgccccagaccttctctgtgctgattggcaacagagagtggctgcggcggaacggcctgaccatctcctccgatgtgtccgacgccatgaccgaccacgagatgaagggccagaccgccattctggtggccattgacggggtgctgtgcggcatgatcgcaatcgccgatgccgtgaaacaggaagcagcactggccgtgcacaccctgcagtctatgggagtggatgtggtgctgatcaccggcgacaacagaaagaccgccagggccattgccacccaggtgggcatcaacaaggtgttcgccgaggtgctgcccagccacaaagtggccaaggtgcaggaactgcagaacaaaggcaaaaaggtggccatggtgggagatggcgtgaacgactctcctgctctggcccaggcagatatgggcgtggccatcggcacaggcaccgacgtggcaattgaggctgctgacgtggtgctgattcggaacgacctgctggacgtggtggcctccatccacctgtccaagagaaccgtgcggcggatcagaatcaacctggtgctggcactgatctataacctcgtgggcatccctatcgccgctggcgtgttcatgcctatcggaatcgtgctgcagccctggatgggctctgccgccatggctgcaagctccgtgtctgtggtgctgtccagcctgcagctgaagtgctacaagaagcccgacctggaaagatacgaggcccaggcccacggacacatgaagcctctgacagcctcccaggtgtccgtgcacatcggcatggacgacagatggcgggacagccctagagccaccccttgggatcaggtgtcatacgtgtcacaggtgtccctgagcagcctgaccagcgacaagcccagcagacatagcgccgctgccgacgacgatggggacaagtggtccctgctgctgaacggccgggatgaggaacagtacatc

SEQ ID NO: 14 - DNA, 4317 bp, synthetic construct
  source 1..4317: mol_type = other DNA; note = Description of Artificial Sequence: Syntheticpolynucleotide
atgcccgagcaggaaagacagatcaccgccagagagggcgccagccggaagatcctgagcaagctgagcctgcccaccagagcctgggagcccgccatgaagaagtccttcgccttcgacaacgtgggctacgagggcggcctggacggactgggaccatcttctcaggtggccacaagcaccgtgcgcatcctgggcatgacctgccagagctgcgtgaagtccatcgaggaccggatcagcaacctgaagggcatcatcagcatgaaggtgtccctggaacagggcagcgccaccgtgaaatacgtgccctctgtcgtgtgcctgcagcaggtgtgccaccagatcggcgacatgggcttcgaggcctctatcgccgagggaaaggccgcctcttggccctctagaagcctgcctgctcaggaagccgtcgtgaagctgcgggtggaagggatgacctgtcagtcctgcgtgtccagcatcgagggcaaagtgcggaagctgcagggcgtggtgcgcgtgaaagtgtctctgagcaaccaggaagctgtgatcacctaccagccctacctgatccagcccgaggacctgagggaccacgtgaacgatatgggatttgaggccgccatcaagagcaaggtggcccctctgtctctgggccccatcgacatcgagagactgcagagcaccaaccccaagcggcctctgagcagcgccaaccagaacttcaacaacagcgagacactgggccaccagggcagccacgtcgtgacactgcagagcatccaggtgtcactggaaaacaagaccgcccaggtgaagtacgaccccagctgcacaagccccgtggccctgcagagagccattgaagctctgccccctggcaacttcaaagtgtccctgcctgacggagccgagggctccggaacagatcacagaagcagcagcagccacagccctggcagcccccctagaaatcaggtgcagggcacctgtagcaccaccctgatcgccattgccggcatgacatgcgccagctgcgtgcactctattgagggcatgatctcccagctggaaggcgtgcagcagatcagtgtgtctctggccgagggcaccgccacagtgctgtacaaccctagcgtgatcagccccgaagaactgagagccgccattgaggacatgggattcgaagccagcgtggtgtccgagagctgctccaccaaccctctgggcaatcacagcgccggcaacagcatggtgcagaccaccgacggcacccccaccagcgtgcaggaagtggccccacatacaggcagactgcccgccaatcacgcccccgatatcctggccaagagcccccagagtacaagagccgtggccccccagaagtgcttcctgcagatcaagggcatgacttgtgcctcttgtgtgtccaatatcgagcggaacctgcagaaagaggccggcgtgctgtctgtgctggtggctctgatggccggcaaggccgagatcaaatacgaccccgaagtgattcagcccctggaaatcgcccagtttatccaggacctgggctttgaagccgccgtgatggaagattacgccggctccgacggcaacatcgagctgaccatcaccggaatgacctgcgcctcctgtgtgcacaacattgagtccaagctgacccggaccaacggcatcacctacgcctctgtggctctggccacctccaaggccctcgtgaagttcgatcccgagatcatcggccccagggacatcatcaagatcatcgaagagatcggcttccacgccagcctggcccagaggaaccctaacgcccaccacctggaccacaagatggaaatcaagcagtggaagaaaagcttcctgtgcagcctggtgttcggcatccccgtgatggccctgatgatctacatgctgatccccagcaacgagccccaccagtccatggtgctggatcacaacatcatccccggcctgtctatcctgaacctgatcttcttcatcctgtgcaccttcgtgcagctgctgggcggctggtacttctacgtgcaggcctacaagtccctgcggcacagatccgccaacatggacgtgctgatcgtgctggccacatctatcgcctacgtgtactccctcgtgatcctggtggtggccgtggccgagaaagccgagagaagccctgtgaccttcttcgacaccccccctatgctgttcgtgtttatcgccctgggccggtggctggaacacctggccaaaagcaagaccagcgaggccctggctaagctgatgagtctgcaggccaccgaggccacagtcgtgaccctgggcgaggacaacctgatcatccgcgaggaacaggtgccaatggaactggtgcagcggggcgacatcgtgaaggtggtgcctggcggcaagttccccgtggacggaaaagtgctggaagggaataccatggccgacgagagcctgatcacaggcgaggccatgcccgtgaccaagaaacctggcagcacagtgatcgccggcagcatcaatgcccacggcagcgtgctgattaaggccacacacgtgggcaacgataccaccctggctcagattgtgaagctggtggaagaggcccagatgagcaaggcccccattcagcagctggctgaccggttcagcggctacttcgtgccctttatcatcatcatgagcaccctgacactggtcgtgtggatcgtgatcggctttatcgacttcggagtggtgcagagatacttccccaaccctaacaagcacatcagccagacagaagtgatcatcagattcgcctttcagaccagcatcaccgtgctgtgtatcgcctgcccctgtagcctgggactggccacacctaccgctgtgatggtgggaacaggcgtggccgctcagaacggcatcctgatcaaggggggcaagcctctggaaatggctcacaagatcaagaccgtgatgttcgacaagaccggcaccatcacccacggcgtgcccagagtgatgagagtgctgctgctgggggatgtggccaccctgcctctgagaaaggtgctggctgtcgtgggcacagccgaggctagctctgaacacccactgggagtggccgtgacaaagtactgcaaagaggaactgggcaccgaaaccctgggctactgcaccgactttcaggccgtgcctggctgtggcatcggctgcaaggtgtccaacgtggaaggcatcctggcccacagcgagaggccactgtctgcccctgccagccacctgaacgaggccggatctctgcccgccgaaaaggacgctgtgccccagaccttctctgtgctgattggcaacagagagtggctgcggcggaacggcctgaccatctcctccgatgtgtccgacgccatgaccgaccacgagatgaagggccagaccgccattctggtggccattgacggggtgctgtgcggcatgatcgcaatcgccgatgccgtgaaacaggaagcagcactggccgtgcacaccctgcagtctatgggagtggatgtggtgctgatcaccggcgacaacagaaagaccgccagggccattgccacccaggtgggcatcaacaaggtgttcgccgaggtgctgcccagccacaaagtggccaaggtgcaggaactgcagaacaaaggcaaaaaggtggccatggtgggagatggcgtgaacgactctcctgctctggcccaggcagatatgggcgtggccatcggcacaggcaccgacgtggcaattgaggctgctgacgtggtgctgattcggaacgacctgctggacgtggtggcctccatccacctgtccaagagaaccgtgcggcggatcagaatcaacctggtgctggcactgatctataacctcgtgggcatccctatcgccgctggcgtgttcatgcctatcggaatcgtgctgcagccctggatgggctctgccgccatggctgcaagctccgtgtctgtggtgctgtccagcctgcagctgaagtgctacaagaagcccgacctggaaagatacgaggcccaggcccacggacacatgaagcctctgacagcctcccaggtgtccgtgcacatcggcatggacgacagatggcgggacagccctagagccaccccttgggatcaggtgtcatacgtgtcacaggtgtccctgagcagcctgaccagcgacaagcccagcagacatagcgccgctgccgacgacgatggggacaagtggtccctgctgctgaacggccgggatgaggaacagtacatc

SEQ ID NO: 15 - DNA, 4395 bp, synthetic construct
  source 1..4395: mol_type = other DNA; note = Description of Artificial Sequence: Syntheticpolynucleotide
atgccagaacaggaacgccagatcacagcaagagagggagcaagtcggaaaatcctgagcaaactgagcctgccaaccagagcatgggaacccgcaatgaagaaaagcttcgcctttgacaacgtgggatacgagggagggctggatggactgggacctagctcccaggtggccacctctacagtccgaatcctgggcatgacttgccagagttgcgtgaaatcaattgaagaccggatcagtaatctgaagggaatcattagcatgaaagtgtccctggagcagggctcagccaccgtgaagtatgtccctagcgtggtctgcctgcagcaggtgtgccaccagatcggcgatatggggttcgaggcctccattgctgaagggaaagccgcttcttggcctagccggtccctgccagcacaggaagcagtggtcaagctgagagtggagggaatgacatgccagagctgcgtgagcagtatcgaaggaaaggtccgaaaactgcagggcgtggtccgggtgaaggtctctctgagtaaccaggaggccgtgattacctaccagccctatctgatccagcctgaagacctgagggatcacgtgaatgacatgggcttcgaggcagccatcaagtccaaagtggccccactgtctctggggcccattgatatcgaaagactgcagtccaccaacccaaagaggcccctgtcaagcgccaaccagaacttcaacaatagtgagaccctgggacaccagggctcacatgtggtcacactgcagctgaggattgacggcatgcactgcaagtcttgcgtgctgaacattgaggaaaatatcggccagctgctgggggtgcagtctatccaggtcagtctggagaacaagactgctcaggtgaaatacgatccttcatgcaccagcccagtggcactgcagcgcgctatcgaagcactgccccctggaaatttcaaggtgagcctgcctgacggagcagagggatccggaaccgatcacaggtcctctagttcacattccccagggtctccaccacgaaaccaggtgcagggaacatgttccaccacactgattgcaatcgccggcatgacttgcgcctcatgcgtgcacagcattgaagggatgatctctcagctggagggagtgcagcagatctcagtcagcctggccgagggcactgctaccgtgctgtacaatcccagtgtcatctcacctgaggaactgcgggctgcaattgaggacatggggttcgaagcttccgtggtctccgaatcttgcagtaccaaccccctggggaatcattccgccggaaactctatggtgcagactaccgacgggacacctacttctgtgcaggaggtcgcaccacacacaggacgcctgccagccaatcatgctcccgatatcctggccaaaagcccccagtccactcgagctgtggcacctcagaagtgttttctgcagatcaaaggcatgacctgcgcctcttgcgtgagcaacattgagcggaatctgcagaaggaagctggggtgctgagcgtgctggtcgcactgatggccggaaaggctgagatcaagtacgaccctgaagtgatccagccactggagattgcccagttcatccaggatctgggctttgaggccgctgtgatggaagactatgctgggagcgatggaaacattgaactgaccatcaccggaatgacttgtgcctcttgcgtgcacaacatcgagagtaaactgactagaaccaatgggattacctacgccagtgtggccctggctacatcaaaggctctggtgaaattcgaccccgagatcattggacctagggatatcattaagatcattgaggaaatcggctttcacgcaagcctggcccagcgcaacccaaatgcccaccatctggaccataagatggagatcaagcagtggaagaaaagtttcctgtgctcactggtgtttggaatccccgtcatggccctgatgatctacatgctgatccctagcaacgagccacaccagtccatggtgctggatcataacatcattcctggcctgtccatcctgaatctgattttctttatcctgtgcacattcgtgcagctgctgggaggctggtacttttatgtgcaggcatataaatcactgcgacaccggagcgccaatatggacgtgctgattgtcctggcaacctctatcgcctacgtgtatagtctggtcatcctggtggtcgcagtggcagagaaggcagaacggagcccagtgactttctttgatacccctccaatgctgttcgtgtttatcgctctgggcagatggctggaacatctggcaaagtcaaaaaccagcgaggctctggcaaagctgatgagcctgcaggctaccgaagcaacagtggtcactctgggagaggacaacctgatcattcgcgaggaacaggtgcctatggaactggtccagcgaggcgatatcgtgaaggtggtcccagggggaaaattccccgtggacggcaaggtcctggaggggaatactatggccgatgaatccctgatcaccggcgaggctatgcctgtgacaaagaaaccaggatcaactgtcattgctggcagcatcaacgcacacgggtccgtgctgatcaaggccacacatgtcgggaatgacacaactctggctcagattgtgaaactggtcgaggaagcccagatgtccaaggctcctatccagcagctggccgatcggttctccggctacttcgtgcccttcatcattatcatgtctacactgactctggtggtctggattgtgatcggattcattgactttggcgtggtccagagatattttcccaaccctaataagcacatcagccagaccgaagtgatcatcaggttcgcatttcagaccagtattacagtgctgtgcatcgcctgcccatgttcactggggctggctacccccacagcagtgatggtcggaacaggagtggcagcacagaacggaattctgatcaagggcgggaaacccctggagatggcccacaagatcaaaactgtgatgtttgacaaaactgggaccattacacatggagtgccccgcgtcatgcgagtgctgctgctgggcgatgtggcaaccctgcctctgagaaaggtcctggcagtggtcggaacagcagaggctagctccgaacacccactgggggtggccgtcacaaagtactgcaaagaggaactgggcactgagaccctggggtattgtactgacttccaggcagtgcccggatgcggaatcggatgtaaagtctctaacgtggaagggattctggctcacagtgagcggcccctgagcgcacctgcatcccatctgaatgaagcaggaagcctgccagcagagaaggacgctgtgcctcagaccttttccgtcctgatcggcaacagagaatggctgcggagaaatgggctgacaatttctagtgacgtgtccgatgccatgacagatcacgagatgaaaggccagactgcaattctggtggccatcgacggagtcctgtgcggcatgattgctatcgcagatgccgtgaagcaggaggctgcactggccgtccataccctgcagtctatgggcgtggacgtggtcctgatcaccggggataaccggaaaacagctagagcaattgccactcaagtgggcatcaataaggtgttcgctgaagtcctgcctagccacaaggtcgcaaaagtgcaggagctgcagaacaagggcaagaaagtcgccatggtgggagacggcgtgaatgatagcccagctctggcacaggcagacatgggagtcgctattgggacaggaactgacgtggcaatcgaggccgctgatgtggtcctgattaggaatgacctgctggatgtggtcgcttctattcatctgagtaagaggacagtgaggcgcattcgcatcaacctggtgctggccctgatctacaatctggtgggaattccaatcgcagccggcgtgtttatgccaattgggatcgtcctgcagccctggatgggctcagctgcaatggccgcttcaagcgtgagcgtggtcctgtcctctctgcagctgaaatgctacaagaaaccagacctggagcggtacgaagctcaggcacacggacatatgaagcccctgaccgcttcccaggtgtctgtccacatcggcatggacgatagatggagggacagcccaagggccactccatgggatcaggtcagttacgtgagccaggtcagcctgagttcactgaccagcgacaagccctcccgccattctgcagccgctgatgacgacggggacaagtggagcctgctgctgaacggaagggacgaagaacagtatatc

SEQ ID NO: 16 - DNA, 3105 bp, synthetic construct
  source 1..3105: mol_type = other DNA; note = Description of Artificial Sequence: Syntheticpolynucleotide
atgcctgagcaggagagacagatcacagccagagaaggggccagtcggaaaatcttatctaagctttctttgcctacccgtgcctgggaaccagcaatgaagaagagttttgcttttgacaatgttggctatgaaggtggtctggatggcctgggcccttcttctcagccgcagaagtgcttcttacagatcaaaggcatgacctgtgcatcctgtgtgtctaacatagaaaggaatctgcagaaagaagctggtgttctctccgtgttggttgccttgatggcaggaaaggcagagatcaagtatgacccagaggtcatccagcccctcgagatagctcagttcatccaggacctgggttttgaggcagcagtcatggaggactacgcaggctccgatggcaacattgagctgacaatcacagggatgacctgcgcgtcctgtgtccacaacatagagtccaaactcacgaggacaaatggcatcacttatgcctccgttgcccttgccaccagcaaagcccttgttaagtttgacccggaaattatcggtccacgggatattatcaaaattattgaggaaattggctttcatgcttccctggcccagagaaaccccaacgctcatcacttggaccacaagatggaaataaagcagtggaagaagtctttcctgtgcagcctggtgtttggcatccctgtcatggccttaatgatctatatgctgatacccagcaacgagccccaccagtccatggtcctggaccacaacatcattccaggactgtccattctaaatctcatcttctttatcttgtgtacctttgtccagctcctcggtgggtggtacttctacgttcaggcctacaaatctctgagacacaggtcagccaacatggacgtgctcatcgtcctggccacaagcattgcttatgtttattctctggtcatcctggtggttgctgtggctgagaaggcggagaggagccctgtgacattcttcgacacgccccccatgctctttgtgttcattgccctgggccggtggctggaacacttggcaaagagcaaaacctcagaagccctggctaaactcatgtctctccaagccacagaagccaccgttgtgacccttggtgaggacaatttaatcatcagggaggagcaagtccccatggagctggtgcagcggggcgatatcgtcaaggtggtccctgggggaaagtttccagtggatgggaaagtcctggaaggcaataccatggctgatgagtccctcatcacaggagaagccatgccagtcactaagaaacccggaagcactgtaattgcggggtctataaatgcacatggctctgtgctcattaaagctacccacgtgggcaatgacaccactttggctcagattgtgaaactggtggaagaggctcagatgtcaaaggcacccattcagcagctggctgaccggtttagtggatattttgtcccatttatcatcatcatgtcaactttgacgttggtggtatggattgtaatcggttttatcgattttggtgttgttcagagatactttcctaaccccaacaagcacatctcccagacagaggtgatcatccggtttgctttccagacgtccatcacggtgctgtgcattgcctgcccctgctccctggggctggccacgcccacggctgtcatggtgggcaccggggtggccgcgcagaacggcatcctcatcaagggaggcaagcccctggagatggcgcacaagataaagactgtgatgtttgacaagactggcaccattacccatggcgtccccagggtcatgcgggtgctcctgctgggggatgtggccacactgcccctcaggaaggttctggctgtggtggggactgcggaggccagcagtgaacaccccttgggcgtggcagtcaccaaatactgtaaagaggaacttggaacagagaccttgggatactgcacggacttccaggcagtgccaggctgtggaattgggtgcaaagtcagcaacgtggaaggcatcctggcccacagtgagcgccctttgagtgcaccggccagtcacctgaatgaggctggcagccttcccgcagaaaaagatgcagtcccccagaccttctctgtgctgattggaaaccgtgagtggctgaggcgcaacggtttaaccatttctagcgatgtcagtgacgctatgacagaccacgagatgaaaggacagacagccatcctggtggctattgacggtgtgctctgtgggatgatcgcaatcgcagacgctgtcaagcaggaggctgccctggctgtgcacacgctgcagagcatgggtgtggacgtggttctgatcacgggggacaaccggaagacagccagagctattgccacccaggttggcatcaacaaagtctttgcagaggtgctgccttcgcacaaggtggccaaggtccaggagctccagaataaagggaagaaagtcgccatggtgggggatggggtcaatgactccccggccttggcccaggcagacatgggtgtggccattggcaccggcacggatgtggccatcgaggcagccgacgtcgtccttatcagaaatgatttgctggatgtggtggctagcattcacctttccaagaggactgtccgaaggatacgcatcaacctggtcctggcactgatttataacctggttgggatacccattgcagcaggtgtcttcatgcccatcggcattgtgctgcagccctggatgggctcagcggccatggcagcctcctctgtgtctgtggtgctctcatccctgcagctcaagtgctataagaagcctgacctggagaggtatgaggcacaggcgcatggccacatgaagcccctgacggcatcccaggtcagtgtgcacataggcatggatgacaggtggcgggactcccccagggccacaccatgggaccaggtcagctatgtcagccaggtgtcgctgtcctccctgacgtccgacaagccatctcggcacagcgctgcagcagacgatgatggggacaagtggtctctgctcctgaatggcagggatgaggagcagtacatc

SEQ ID NO: 17 - DNA, 3105 bp, synthetic construct
  source 1..3105: mol_type = other DNA; note = Description of Artificial Sequence: Syntheticpolynucleotide
atgccagaacaggaacgccagatcacagcaagagagggagcaagtcggaaaatcctgagcaaactgagcctgccaaccagagcatgggaacccgcaatgaagaaaagcttcgcctttgacaacgtgggatacgagggagggctggatggactgggacctagctcccagcctcagaagtgttttctgcagatcaaaggcatgacctgcgcctcttgcgtgagcaacattgagcggaatctgcagaaggaagctggggtgctgagcgtgctggtcgcactgatggccggaaaggctgagatcaagtacgaccctgaagtgatccagccactggagattgcccagttcatccaggatctgggctttgaggccgctgtgatggaagactatgctgggagcgatggaaacattgaactgaccatcaccggaatgacttgtgcctcttgcgtgcacaacatcgagagtaaactgactagaaccaatgggattacctacgccagtgtggccctggctacatcaaaggctctggtgaaattcgaccccgagatcattggacctagggatatcattaagatcattgaggaaatcggctttcacgcaagcctggcccagcgcaacccaaatgcccaccatctggaccataagatggagatcaagcagtggaagaaaagtttcctgtgctcactggtgtttggaatccccgtcatggccctgatgatctacatgctgatccctagcaacgagccacaccagtccatggtgctggatcataacatcattcctggcctgtccatcctgaatctgattttctttatcctgtgcacattcgtgcagctgctgggaggctggtacttttatgtgcaggcatataaatcactgcgacaccggagcgccaatatggacgtgctgattgtcctggcaacctctatcgcctacgtgtatagtctggtcatcctggtggtcgcagtggcagagaaggcagaacggagcccagtgactttctttgatacccctccaatgctgttcgtgtttatcgctctgggcagatggctggaacatctggcaaagtcaaaaaccagcgaggctctggcaaagctgatgagcctgcaggctaccgaagcaacagtggtcactctgggagaggacaacctgatcattcgcgaggaacaggtgcctatggaactggtccagcgaggcgatatcgtgaaggtggtcccagggggaaaattccccgtggacggcaaggtcctggaggggaatactatggccgatgaatccctgatcaccggcgaggctatgcctgtgacaaagaaaccaggatcaactgtcattgctggcagcatcaacgcacacgggtccgtgctgatcaaggccacacatgtcgggaatgacacaactctggctcagattgtgaaactggtcgaggaagcccagatgtccaaggctcctatccagcagctggccgatcggttctccggctacttcgtgcccttcatcattatcatgtctacactgactctggtggtctggattgtgatcggattcattgactttggcgtggtccagagatattttcccaaccctaataagcacatcagccagaccgaagtgatcatcaggttcgcatttcagaccagtattacagtgctgtgcatcgcctgcccatgttcactggggctggctacccccacagcagtgatggtcggaacaggagtggcagcacagaacggaattctgatcaagggcgggaaacccctggagatggcccacaagatcaaaactgtgatgtttgacaaaactgggaccattacacatggagtgccccgcgtcatgcgagtgctgctgctgggcgatgtggcaaccctgcctctgagaaaggtcctggcagtggtcggaacagcagaggctagctccgaacacccactgggggtggccgtcacaaagtactgcaaagaggaactgggcactgagaccctggggtattgtactgacttccaggcagtgcccggatgcggaatcggatgtaaagtctctaacgtggaagggattctggctcacagtgagcggcccctgagcgcacctgcatcccatctgaatgaagcaggaagcctgccagcagagaaggacgctgtgcctcagaccttttccgtcctgatcggcaacagagaatggctgcggagaaatgggctgacaatttctagtgacgtgtccgatgccatgacagatcacgagatgaaaggccagactgcaattctggtggccatcgacggagtcctgtgcggcatgattgctatcgcagatgccgtgaagcaggaggctgcactggccgtccataccctgcagtctatgggcgtggacgtggtcctgatcaccggggataaccggaaaacagctagagcaattgccactcaagtgggcatcaataaggtgttcgctgaagtcctgcctagccacaaggtcgcaaaagtgcaggagctgcagaacaagggcaagaaagtcgccatggtgggagacggcgtgaatgatagcccagctctggcacaggcagacatgggagtcgctattgggacaggaactgacgtggcaatcgaggccgctgatgtggtcctgattaggaatgacctgctggatgtggtcgcttctattcatctgagtaagaggacagtgaggcgcattcgcatcaacctggtgctggccctgatctacaatctggtgggaattccaatcgcagccggcgtgtttatgccaattgggatcgtcctgcagccctggatgggctcagctgcaatggccgcttcaagcgtgagcgtggtcctgtcctctctgcagctgaaatgctacaagaaaccagacctggagcggtacgaagctcaggcacacggacatatgaagcccctgaccgcttcccaggtgtctgtccacatcggcatggacgatagatggagggacagcccaagggccactccatgggatcaggtcagttacgtgagccaggtcagcctgagttcactgaccagcgacaagccctcccgccattctgcagccgctgatgacgacggggacaagtggagcctgctgctgaacggaagggacgaagaacagtatatc

SEQ ID NO: 18 - DNA, 3963 bp, synthetic construct
  source 1..3963: mol_type = other DNA; note = Description of Artificial Sequence: Syntheticpolynucleotide
atgcctgagcaggagagacagatcacagccagagaaggggccagtcggaaaatcttatctaagctttctttgcctacccgtgcctgggaaccagcaatgaagaagagttttgcttttgacaatgttggctatgaaggtggtctggatggcctgggcccttcttctcaggtggccaccagcacagtcaggatcttgggcatgacttgccagtcatgtgtgaagtccattgaggacaggatttccaatttgaaaggcatcatcagcatgaaggtttccctggaacaaggcagtgccactgtgaaatatgtgccatcggttgtgtgcctgcaacaggtttgccatcaaattggggacatgggcttcgaggccagcattgcagaaggaaaggcagcctcctggccctcaaggtccttgcctgcccaggaggctgtggtcaagctccgggtggagggcatgacctgccagtcctgtgtcagctccattgaaggcaaggtccggaaactgcaaggagtagtgagagtcaaagtctcactcagcaaccaagaggccgtcatcacttatcagccttatctcattcagcccgaagacctcagggaccatgtaaatgacatgggatttgaagctgccatcaagagcaaagtggctcccttaagcctgggaccaattggcatgacctgtgcatcctgtgtccattccattgaaggcatgatctcccaactggaaggggtgcagcaaatatcggtgtctttggccgaagggactgcaacagttctttataatccctctgtaattagcccagaagaactcagagctgctatagaagacatgggatttgaggcttcagtcgtttctgaaagctgttctactaaccctcttggaaaccacagtgctgggaattccatggtgcaaactacagatggtacacctacatctgtgcaggaagtggctccccacactgggaggctccctgcaaaccatgccccggacatcttggcaaagtccccacaatcaaccagagcagtggcaccgcagaagtgcttcttacagatcaaaggcatgacctgtgcatcctgtgtgtctaacatagaaaggaatctgcagaaagaagctggtgttctctccgtgttggttgccttgatggcaggaaaggcagagatcaagtatgacccagaggtcatccagcccctcgagatagctcagttcatccaggacctgggttttgaggcagcagtcatggaggactacgcaggctccgatggcaacattgagctgacaatcacagggatgacctgcgcgtcctgtgtccacaacatagagtccaaactcacgaggacaaatggcatcacttatgcctccgttgcccttgccaccagcaaagcccttgttaagtttgacccggaaattatcggtccacgggatattatcaaaattattgaggaaattggctttcatgcttccctggcccagagaaaccccaacgctcatcacttggaccacaagatggaaataaagcagtggaagaagtctttcctgtgcagcctggtgtttggcatccctgtcatggccttaatgatctatatgctgatacccagcaacgagccccaccagtccatggtcctggaccacaacatcattccaggactgtccattctaaatctcatcttctttatcttgtgtacctttgtccagctcctcggtgggtggtacttctacgttcaggcctacaaatctctgagacacaggtcagccaacatggacgtgctcatcgtcctggccacaagcattgcttatgtttattctctggtcatcctggtggttgctgtggctgagaaggcggagaggagccctgtgacattcttcgacacgccccccatgctctttgtgttcattgccctgggccggtggctggaacacttggcaaagagcaaaacctcagaagccctggctaaactcatgtctctccaagccacagaagccaccgttgtgacccttggtgaggacaatttaatcatcagggaggagcaagtccccatggagctggtgcagcggggcgatatcgtcaaggtggtccctgggggaaagtttccagtggatgggaaagtcctggaaggcaataccatggctgatgagtccctcatcacaggagaagccatgccagtcactaagaaacccggaagcactgtaattgcggggtctataaatgcacatggctctgtgctcattaaagctacccacgtgggcaatgacaccactttggctcagattgtgaaactggtggaagaggctcagatgtcaaaggcacccattcagcagctggctgaccggtttagtggatattttgtcccatttatcatcatcatgtcaactttgacgttggtggtatggattgtaatcggttttatcgattttggtgttgttcagagatactttcctaaccccaacaagcacatctcccagacagaggtgatcatccggtttgctttccagacgtccatcacggtgctgtgcattgcctgcccctgctccctggggctggccacgcccacggctgtcatggtgggcaccggggtggccgcgcagaacggcatcctcatcaagggaggcaagcccctggagatggcgcacaagataaagactgtgatgtttgacaagactggcaccattacccatggcgtccccagggtcatgcgggtgctcctgctgggggatgtggccacactgcccctcaggaaggttctggctgtggtggggactgcggaggccagcagtgaacaccccttgggcgtggcagtcaccaaatactgtaaagaggaacttggaacagagaccttgggatactgcacggacttccaggcagtgccaggctgtggaattgggtgcaaagtcagcaacgtggaaggcatcctggcccacagtgagcgccctttgagtgcaccggccagtcacctgaatgaggctggcagccttcccgcagaaaaagatgcagtcccccagaccttctctgtgctgattggaaaccgtgagtggctgaggcgcaacggtttaaccatttctagcgatgtcagtgacgctatgacagaccacgagatgaaaggacagacagccatcctggtggctattgacggtgtgctctgtgggatgatcgcaatcgcagacgctgtcaagcaggaggctgccctggctgtgcacacgctgcagagcatgggtgtggacgtggttctgatcacgggggacaaccggaagacagccagagctattgccacccaggttggcatcaacaaagtctttgcagaggtgctgccttcgcacaaggtggccaaggtccaggagctccagaataaagggaagaaagtcgccatggtgggggatggggtcaatgactccccggccttggcccaggcagacatgggtgtggccattggcaccggcacggatgtggccatcgaggcagccgacgtcgtccttatcagaaatgatttgctggatgtggtggctagcattcacctttccaagaggactgtccgaaggatacgcatcaacctggtcctggcactgatttataacctggttgggatacccattgcagcaggtgtcttcatgcccatcggcattgtgctgcagccctggatgggctcagcggccatggcagcctcctctgtgtctgtggtgctctcatccctgcagctcaagtgctataagaagcctgacctggagaggtatgaggcacaggcgcatggccacatgaagcccctgacggcatcccaggtcagtgtgcacataggcatggatgacaggtggcgggactcccccagggccacaccatgggaccaggtcagctatgtcagccaggtgtcgctgtcctccctgacgtccgacaagccatctcggcacagcgctgcagcagacgatgatggggacaagtggtctctgctcctgaatggcagggatgaggagcagtacatc

SEQ ID NO: 19 - DNA, 56 bp, synthetic construct
  source 1..56: mating_type = Description of Artificial Sequence: Syntheticpolynucleotide; mol_type = other DNA
gtaaggtaagaattgaatttctcagttgaaggatgcttacactcttgtccatctag

SEQ ID NO: 20 - DNA, 49 bp, synthetic construct
  source 1..49: mol_type = other DNA; note = Description of Artificial Sequence: Syntheticoligonucleotide
gtgtgtatgctcaggggctgggaaaggaggggagggagctccggctcag

SEQ ID NO: 21 - DNA, 266 bp, synthetic construct
  source 1..266: mol_type = other DNA; note = Description of Artificial Sequence: Syntheticpolynucleotide
gtgatgcggttttggcagtacatcaatgggcgtggatagcggtttgactcacggggatttccaagtctccaccccattgacgtcaatgggagtttgttttggcaccaaaatcaacgggactttccaaaatgtcgtaacaactccgccccattgacgcaaatgggcggtaggcgtgtacggtgggaggtctatataagcagagctggtaccgtaaggtaagaattgaatttctcagttgaaggatgcttacactcttgtccatctag

SEQ ID NO: 22 - DNA, 259 bp, synthetic construct
  source 1..259: mol_type = other DNA; note = Description of Artificial Sequence: Syntheticpolynucleotide
gtgatgcggttttggcagtacatcaatgggcgtggatagcggtttgactcacggggatttccaagtctccaccccattgacgtcaatgggagtttgttttggcaccaaaatcaacgggactttccaaaatgtcgtaacaactccgccccattgacgcaaatgggcggtaggcgtgtacggtgggaggtctatataagcagagctggtaccgtgtgtatgctcaggggctgggaaaggaggggagggagctccggctcag

SEQ ID NO: 23 - DNA, 117 bp, synthetic construct
  source 1..117: mol_type = other DNA; note = Description of Artificial Sequence: Syntheticpolynucleotide
gtgatgacgtgtcccataaggcccctcggtctaaggcttccctatttcctggttcgccggcggccattttgggtggaagcgatagctgagtggcggcggctgctgattgtgttctag

SEQ ID NO: 24 - DNA, 117 bp, synthetic construct
  source 1..117: mol_type = other DNA; note = Description of Artificial Sequence: Syntheticpolynucleotide
gtgatgacgtgtcccatacttccgggtcaggtgggccggctgtcttgaccttctttgcggctcggccattttgtcccagtcagtccggaggctgcggctgcagaagtaccgcctgcg

SEQ ID NO: 25 - DNA, 117 bp, synthetic construct
  source 1..117: mol_type = other DNA; note = Description of Artificial Sequence: Syntheticpolynucleotide
gtgatgacgtgtcccatattttcatctcgcgagacttgtgagcggccatcttggtcctgccctgacagattctcctatcggggtcacagggacgctaagattgctacctggactttc

SEQ ID NO: 26 - DNA, 117 bp, synthetic construct
  source 1..117: mol_type = other DNA; note = Description of Artificial Sequence: Syntheticpolynucleotide
gtgatgacgtgtcccatggcctcattggatgagaggtcccacctcacggcccgaggcggggcttctttgcgcttaaaagccgagccgggccaatgttcaaatgcgcagctcttagtc

SEQ ID NO: 27 - DNA, 117 bp, synthetic construct
  source 1..117: mol_type = other DNA; note = Description of Artificial Sequence: Syntheticpolynucleotide
gtgatgacgtgtcccatcccccctccaccccctagcccgcggagcacgctgggatttggcgcccccctcctcggtgcaacctatataaggctcacagtctgcgctcctggtacacgc

SEQ ID NO: 28 - DNA, 100 bp, synthetic construct
  source 1..100: mol_type = other DNA; note = Description of Artificial Sequence: Syntheticpolynucleotide
cccccctccaccccctagcccgcggagcacgctgggatttggcgcccccctcctcggtgcaacctatataaggctcacagtctgcgctcctggtacacgc

SEQ ID NO: 29 - DNA, 100 bp, synthetic construct
  source 1..100: mol_type = other DNA; note = Description of Artificial Sequence: Syntheticpolynucleotide
ggcctcattggatgagaggtcccacctcacggcccgaggcggggcttctttgcgcttaaaagccgagccgggccaatgttcaaatgcgcagctcttagtc

SEQ ID NO: 30 - DNA, 100 bp, synthetic construct
  source 1..100: mol_type = other DNA; note = Description of Artificial Sequence: Syntheticpolynucleotide
gggtggggcccgcgcgtataaagggggcgcaggcgggctgggcgttccacaggccaagtgcgctgtgctcgaggggtgccggccaggcctgagcgagcga

SEQ ID NO: 31 - DNA, 100 bp, synthetic construct
  source 1..100: mol_type = other DNA; note = Description of Artificial Sequence: Syntheticpolynucleotide
ggtgcgatattcggattggctggagtcggccatcacgctccagctacgccacttccttttcgtggcactataaagggtgctgcacggcgcttgcatctct

SEQ ID NO: 32 - DNA, 100 bp, synthetic construct
  source 1..100: mol_type = other DNA; note = Description of Artificial Sequence: Syntheticpolynucleotide
acttccgggtcaggtgggccggctgtcttgaccttctttgcggctcggccattttgtcccagtcagtccggaggctgcggctgcagaagtaccgcctgcg

SEQ ID NO: 33 - DNA, 100 bp, synthetic construct
  source 1..100: mol_type = other DNA; note = Description of Artificial Sequence: Syntheticpolynucleotide
gctgagcgcgcgcgatggggcgggaggtttggggtcaaggagcaaactctgcacaagatggcggcggtagcggcagtggcggcgcgtaggaggcggtgag

SEQ ID NO: 34 - DNA, 100 bp, synthetic construct
  source 1..100: mol_type = other DNA; note = Description of Artificial Sequence: Syntheticpolynucleotide
attttcatctcgcgagacttgtgagcggccatcttggtcctgccctgacagattctcctatcggggtcacagggacgctaagattgctacctggactttc

SEQ ID NO: 35 - DNA, 100 bp, synthetic construct
  source 1..100: mol_type = other DNA; note = Description of Artificial Sequence: Syntheticpolynucleotide
tgggacccccggaaggcggaagttctagggcggaagtggccgagaggagaggagaatggcggcggaaggctggatttggcgttggggctggggccggcgg

SEQ ID NO: 36 - DNA, 100 bp, synthetic construct
  source 1..100: mol_type = other DNA; note = Description of Artificial Sequence: Syntheticpolynucleotide
aaggcccctcggtctaaggcttccctatttcctggttcgccggcggccattttgggtggaagcgatagctgagtggcggcggctgctgattgtgttctag

SEQ ID NO: 37 - DNA, 100 bp, synthetic construct
  source 1..100: mol_type = other DNA; note = Description of Artificial Sequence: Syntheticpolynucleotide
agtgacccggaagtagaagtggcccttgcaggcaagagtgctggagggcggcagcggcgaccggagcggtaggagcagcaatttatccgtgtgcagcccc

SEQ ID NO: 38 - DNA, 100 bp, synthetic construct
  source 1..100: mol_type = other DNA; note = Description of Artificial Sequence: Syntheticpolynucleotide
gggaggggcgcgctggggagcttcggcgcatgcgcgctgaggcctgcctgaccgaccttcagcagggctgtggctaccatgttctctcgcgcgggtgtcg

SEQ ID NO: 39 - DNA, 100 bp, synthetic construct
  source 1..100: mol_type = other DNA; note = Description of Artificial Sequence: Syntheticpolynucleotide
actgcgcacgcgcgcggtcgcaccgattcacgcccccttccggcgcctagagcaccgctgccgccatgttgagggggggaccgcgaccagctgggcccct

SEQ ID NO: 40 - DNA, 100 bp, synthetic construct
  source 1..100: mol_type = other DNA; note = Description of Artificial Sequence: Syntheticpolynucleotide
ccctcgaggggcggagcaaaaagtgaggcagcaacgcctccttatcctcgctcccgctttcagttctcaataaggtccgatgttcgtgtataaatgctcg

SEQ ID NO: 41 - DNA, 100 bp, synthetic construct
  source 1..100: mol_type = other DNA; note = Description of Artificial Sequence: Syntheticpolynucleotide
cttggtgaccaaatttgaaaaaaaaaaaaaaccgcgccaactcatgttgttttcaatcaggtccgccaagtttgtatttaaggaactgtttcagttcata

SEQ ID NO: 42 - DNA, 100 bp, synthetic construct
  source 1..100: mol_type = other DNA; note = Description of Artificial Sequence: Syntheticpolynucleotide
ggctgagctatcctattggctatcgggacaaaatttgcttgagccaatcaaagtgctccgtggacaatcgccgttctgtctataaaaaggtgaagcagcg

SEQ ID NO: 43 - DNA, 100 bp, synthetic construct
  source 1..100: mol_type = other DNA; note = Description of Artificial Sequence: Syntheticpolynucleotide
ggaagtgccagaccggaggtgcgtcattcaccggcgacgccgatacggttcctccaccgaggcccatgcgaagctttccactatggcttccagcactgtc

SEQ ID NO: 44 - DNA, 20 bp, synthetic construct
  source 1..20: mol_type = other DNA; note = Description of Artificial Sequence: Syntheticprimer
accacagtccatgccatcac

SEQ ID NO: 45 - DNA, 20 bp, synthetic construct
  source 1..20: mol_type = other DNA; note = Description of Artificial Sequence: Syntheticprimer
tccaccaccctgttgctgta

SEQ ID NO: 46 - DNA, 20 bp, synthetic construct
  source 1..20: mol_type = other DNA; note = Description of Artificial Sequence: Syntheticprimer
gctaccccgaccacatgaag

SEQ ID NO: 47 - DNA, 20 bp, synthetic construct
  source 1..20: mol_type = other DNA; note = Description of Artificial Sequence: Syntheticprimer
tcttgtagttgccgtcgtcc

SEQ ID NO: 48 - DNA, 80 bp, synthetic construct
  source 1..80: mol_type = other DNA; note = Description of Artificial Sequence: Syntheticoligonucleotide
gtacttatataagggggtgggggcgcgttcgtcctcagtcgcgatcgaacactcgagccgagcagacgtgcctacggacc

SEQ ID NO: 49 - DNA, 279 bp, synthetic construct
  source 1..279: mol_type = other DNA; note = Description of Artificial Sequence: Syntheticpolynucleotide
ggggaggctgctggtgaatattaaccaaggtcaccccagttatcggaggagcaaacaggggctaagtccacgctagcgtctgtctgcacatttcgtagagcgagtgttccgatactctaatctccctaggcaaggttcatatttgtgtaggttacttattctccttttgttgactaagtcaataatcagaatcagcaggtttggagtcagcttggcagggatcagcagcctgggttggaaggagggggtataaaagccccttcaccaggagaagccgtc

SEQ ID NO: 50 - DNA, 262 bp, synthetic construct
  source 1..262: mol_type = other DNA; note = Description of Artificial Sequence: Syntheticpolynucleotide
gtttgctgcttgcaatgtttgcccattttagggtggacacaggacgctgtggtttctgagccagggctagcgggcgactcagatcccagccagtggacttagcccctgtttgctcctccgataactggggtgaccttggttaatattcaccagcagcctcccccgttgcccctctggatccactgcttaaatacggacgaggacagggccctgtctcctcagcttcaggcaccaccactgacctgggacagtgaatcgccac

SEQ ID NO: 51 - DNA, 203 bp, synthetic construct
  source 1..203: mol_type = other DNA; note = Description of Artificial Sequence: Syntheticpolynucleotide
tgatgcggttttggcagtacatcaatgggcgtggatagcggtttgactcacggggatttccaagtctccaccccattgacgtcaatgggagtttgttttggcaccaaaatcaacgggactttccaaaatgtcgtaacaactccgccccattgacgcaaatgggcggtaggcgtgtacggtgggaggtctatataagcagagct

SEQ ID NO: 52 - DNA, 251 bp, synthetic construct
  source 1..251: mol_type = other DNA; note = Description of Artificial Sequence: Syntheticpolynucleotide
gtttgctgcttgcaatgtttgcccattttagggtggacacaggacgctgtggtttctgagccagggggcgactcagatcccagccagtggacttagcccctgtttgctcctccgataactggggtgaccttggttaatattcaccagcagcctcccccgttgcccctctggatccactgcttaaatacggacgaggacagggccctgtctcctcagcttcaggcaccaccactgacctgggacagtgaatc

SEQ ID NO: 53 - DNA, 304 bp, synthetic construct
  source 1..304: mol_type = other DNA; note = Description of Artificial Sequence: Syntheticpolynucleotide
cgttacataacttacggtaaatggcccgcctggctgaccgcccaacgacccccgcccattgacgtcaataatgacgtatgttcccatagtaacgccaatagggactttccattgacgtcaatgggtggagtatttacggtaaactgcccacttggcagtacatcaagtgtatcatatgccaagtacgccccctattgacgtcaatgacggtaaatggcccgcctggcattatgcccagtacatgaccttatgggactttcctacttggcagtacatctacgtattagtcatcgctattaccatg

SEQ ID NO: 54 - DNA, 1643 bp, synthetic construct
  source 1..1643: mol_type = other DNA; note = Description of Artificial Sequence: Syntheticpolynucleotide
gttacataacttacggtaaatggcccgcctggctgaccgcccaacgacccccgcccattgacgtcaataatgacgtatgttcccatagtaacgccaatagggactttccattgacgtcaatgggtggagtatttacggtaaactgcccacttggcagtacatcaagtgtatcatatgccaagtacgccccctattgacgtcaatgacggtaaatggcccgcctggcattatgcccagtacatgaccttatgggactttcctacttggcagtacatctacgtattagtcatcgctattaccatgggtcgaggtgagccccacgttctgcttcactctccccatctcccccccctccccacccccaattttgtatttatttattttttaattattttgtgcagcgatgggggcggggggggggggggcgcgcgccaggcggggcggggcggggcgaggggcggggcggggcgaggcggagaggtgcggcggcagccaatcagagcggcgcgctccgaaagtttccttttatggcgaggcggcggcggcggcggccctataaaaagcgaagcgcgcggcgggcgggagtcgctgcgttgccttcgccccgtgccccgctccgcgccgcctcgcgccgcccgccccggctctgactgaccgcgttactcccacaggtgagcgggcgggacggcccttctcctccgggctgtaattagcgcttggtttaatgacggctcgtttcttttctgtggctgcgtgaaagccttaaagggctccgggagggccctttgtgcgggggggagcggctcggggggtgcgtgcgtgtgtgtgtgcgtggggagcgccgcgtgcggcccgcgctgcccggcggctgtgagcgctgcgggcgcggcgcggggctttgtgcgctccgcgtgtgcgcgaggggagcgcggccgggggcggtgccccgcggtgcgggggggctgcgaggggaacaaaggctgcgtgcggggtgtgtgcgtgggggggtgagcagggggtgtgggcgcggcggtcgggctgtaacccccccctgcacccccctccccgagttgctgagcacggcccggcttcgggtgcggggctccgtgcggggcgtggcgcggggctcgccgtgccgggcggggggtggcggcaggtgggggtgccgggcggggcggggccgcctcgggccggggagggctcgggggaggggcgcggcggccccggagcgccggcggctgtcgaggcgcggcgagccgcagccattgccttttatggtaatcgtgcgagagggcgcagggacttcctttgtcccaaatctggcggagccgaaatctgggaggcgccgccgcaccccctctagcgggcgcgggcgaagcggtgcggcgccggcaggaaggaaatgggcggggagggccttcgtgcgtcgccgcgccgccgtccccttctccatctccagcctcggggctgccgcagggggacggctgccttcgggggggacggggcagggcggggttcggcttctggcgtgtgaccggcggctctagagcctctgctaaccatgttcatgccttcttctttttcctacagctcctgggcaacgtgctggttgttgtgctgtctcatcattttggcaaagaatt

SEQ ID NO: 55 - DNA, 231 bp, synthetic construct
  source 1..231: mol_type = other DNA; note = Description of Artificial Sequence: Syntheticpolynucleotide
gctccggtgcccgtcagtgggcagagcgcacatcgcccacagtccccgagaagttggggggaggggtcggcaattgaaccggtgcctagagaaggtggcgcggggtaaactgggaaagtgatgtcgtgtactggctccgcctttttcccgagggtgggggagaaccgtatataagtgcagtagtcgccgtgaacgttctttttcgcaacgggtttgccgccagaacacagg

SEQ ID NO: 56 - DNA, 21 bp, synthetic construct
  source 1..21: mol_type = other DNA; note = Description of Artificial Sequence: Syntheticprimer
gacctttatcttctgctaacc

SEQ ID NO: 57 - DNA, 19 bp, synthetic construct
  source 1..19: mol_type = other DNA; note = Description of Artificial Sequence: Syntheticprimer
caagacgcaagacttacaa

SEQ ID NO: 58 - DNA, 19 bp, synthetic construct
  source 1..19: mol_type = other DNA; note = Description of Artificial Sequence: Syntheticprimer
agggtacatgcagtaccac

SEQ ID NO: 59 - DNA, 20 bp, synthetic construct
  source 1..20: mol_type = other DNA; note = Description of Artificial Sequence: Syntheticprimer
ggcttataacggatggattg

SEQ ID NO: 60 - DNA, 19 bp, synthetic construct
  source 1..19: mol_type = other DNA; note = Description of Artificial Sequence: Syntheticprimer
caccagcaccgtgagaatc

SEQ ID NO: 61 - DNA, 20 bp, synthetic construct
  source 1..20: mol_type = other DNA; note = Description of Artificial Sequence: Syntheticprimer
ccttcatagagatgatgccc

SEQ ID NO: 62 - DNA, 19 bp, synthetic construct
  source 1..19: mol_type = other DNA; note = Description of Artificial Sequence: Syntheticprimer
caccagcaccgtgagaatc

SEQ ID NO: 63 - DNA, 21 bp, synthetic construct
  source 1..21: mol_type = other DNA; note = Description of Artificial Sequence: Syntheticprimer
caccttcatagagatgattcc

SEQ ID NO: 64 - DNA, 21 bp, synthetic construct
  source 1..21: mol_type = other DNA; note = Description of Artificial Sequence: Syntheticprimer
cattccaggactgtccattct

SEQ ID NO: 65 - DNA, 21 bp, synthetic construct
  source 1..21: mol_type = other DNA; note = Description of Artificial Sequence: Syntheticprimer
ggcctgaacgtagaagtacca

SEQ ID NO: 66 - DNA, 100 bp, synthetic construct
  source 1..100: mol_type = other DNA; note = Description of Artificial Sequence: Syntheticpolynucleotide
taatcagtaaccgtcccacaggggatcatactttggaatagcaaatatttgctgaaggttctgggctgcaaagctgaagctttggtttctgctctaaatg

SEQ ID NO: 67 - DNA, 100 bp, synthetic construct
  source 1..100: mol_type = other DNA; note = Description of Artificial Sequence: Syntheticpolynucleotide
tgcagaggcggaaccaggatgtgacgtaataaccgcgcgcggcgctcggcgttcccgcaaggtcgctttgcagagcgggagcgcgcttaagtaactagtc

SEQ ID NO: 68 - DNA, 117 bp, synthetic construct
  source 1..117: mol_type = other DNA; note = Description of Artificial Sequence: Syntheticpolynucleotide
gtgatgacgtgtcccatgctgagcgcgcgcgatggggcgggaggtttggggtcaaggagcaaactctgcacaagatggcggcggtagcggcagtggcggcgcgtaggaggcggtgag

SEQ ID NO: 69 - DNA, 202 bp, synthetic construct
  source 1..202: mol_type = other DNA; note = Description of Artificial Sequence: Syntheticpolynucleotide
gtctgtctgcacatttcgtagagcgagtgttccgatactctaatctccctaggcaaggttcatatttgtgtaggttacttattctccttttgttgactaagtcaataatcagaatcagcaggtttggagtcagcttggcagggatcagcagcctgggttggaaggagggggtataaaagccccttcaccaggagaagccgtc

SEQ ID NO: 70 - DNA, 305 bp, synthetic construct
  source 1..305: mol_type = other DNA; note = Description of Artificial Sequence: Syntheticpolynucleotide
cgccaccccctccaccttggacacaggacgctgtggtttctgagccaggtacaatgactcctttcggtaagtgcagtggaagctgtacactgcccaggcaaagcgtccgggcagcgtaggcgggcgactcagatcccagccagtggacttagcccctgtttgctcctccgataactggggtgaccttggttaatattcaccagcagcctcccccgttgcccctctggatccactgcttaaatacggacgaggacagggccctgtctcctcagcttcaggcaccaccactgacctgggacagtgaa

SEQ ID NO: 71 - DNA, 18 bp, synthetic construct
  source 1..18: mol_type = other DNA; note = Description of Artificial Sequence: Syntheticprimer
aacatcatccctggcctg

SEQ ID NO: 72 - DNA, 20 bp, synthetic construct
  source 1..20: mol_type = other DNA; note = Description of Artificial Sequence: Syntheticprimer
ccaggctatacacgtaggcg

SEQ ID NO: 73 - DNA, 20 bp, synthetic construct
  source 1..20: mol_type = other DNA; note = Description of Artificial Sequence: Syntheticprimer
gtgatggaggactatgccgg

SEQ ID NO: 74 - DNA, 20 bp, synthetic construct
  source 1..20: mol_type = other DNA; note = Description of Artificial Sequence: Syntheticprimer
ttctggtcagcttgctctcg

SEQ ID NO: 75 - DNA, 29 bp, synthetic construct
  source 1..29: mol_type = other DNA; note = Description of Artificial Sequence: Syntheticprobe
tggcaacatcgagctgaccatcacaggca

SEQ ID NO: 76 - DNA, 16 bp, synthetic construct
  source 1..16: mol_type = other DNA; note = Description of Artificial Sequence: Syntheticprimer
tggtgcagctggtctt

SEQ ID NO: 77 - DNA, 18 bp, synthetic construct
  source 1..18: mol_type = other DNA; note = Description of Artificial Sequence: Syntheticprimer
accagcttcacccttgtc

SEQ ID NO: 78 - DNA, 17 bp, synthetic construct
  source 1..17: mol_type = other DNA; note = Description of Artificial Sequence: Syntheticprimer
ctacacctgctcctgtg

SEQ ID NO: 79 - DNA, 17 bp, synthetic construct
  source 1..17: mol_type = other DNA; note = Description of Artificial Sequence: Syntheticprimer
ccggatagccacccatt

SEQ ID NO: 80 - DNA, 17 bp, synthetic construct
  source 1..17: mol_type = other DNA; note = Description of Artificial Sequence: Syntheticprimer
cagcttccaaggaccaa

SEQ ID NO: 81 - DNA, 17 bp, synthetic construct
  source 1..17: mol_type = other DNA; note = Description of Artificial Sequence: Syntheticprimer
cttgcttgccaggttca

SEQ ID NO: 82 - DNA, 18 bp, synthetic construct
  source 1..18: mol_type = other DNA; note = Description of Artificial Sequence: Syntheticprimer
tatttctgggcttggacg

SEQ ID NO: 83 - DNA, 17 bp, synthetic construct
  source 1..17: mol_type = other DNA; note = Description of Artificial Sequence: Syntheticprimer
ccctcccggtaagatct

SEQ ID NO: 84 - DNA, 18 bp, synthetic construct
  source 1..18: mol_type = other DNA; note = Description of Artificial Sequence: Syntheticprimer
cgaatccatgatggggag

SEQ ID NO: 85 - DNA, 17 bp, synthetic construct
  source 1..17: mol_type = other DNA; note = Description of Artificial Sequence: Syntheticprimer
cagtactcgccatcagc

SEQ ID NO: 86 - DNA, 18 bp, synthetic construct
  source 1..18: mol_type = other DNA; note = Description of Artificial Sequence: Syntheticprimer
ctctgggaaatcgtggaa

SEQ ID NO: 87 - DNA, 20 bp, synthetic construct
  source 1..20: mol_type = other DNA; note = Description of Artificial Sequence: Syntheticprimer
ccaggtagctatggtactcc

SEQ ID NO: 88 - DNA, 18 bp, synthetic construct
  source 1..18: mol_type = other DNA; note = Description of Artificial Sequence: Syntheticprimer
catgttcaccggcaacaa

SEQ ID NO: 89 - DNA, 18 bp, synthetic construct
  source 1..18: mol_type = other DNA; note = Description of Artificial Sequence: Syntheticprimer
gccgtaggttctggaact

SEQ ID NO: 90 - protein, 5 aa, Homo sapiens
SEHPL

SEQ ID NO: 91 - protein, 4 aa, Homo sapiens
DKTG

SEQ ID NO: 92 - protein, 7 aa, synthetic construct
  source 1..7: note = Description of Artificial Sequence: Syntheticpeptide
GMXCXXC